European Patent Specification EP 3 666 288 B1, published September 27, 2023. Title: ANTI-MUTATED KRAS T CELL RECEPTORS. Applicant: THE UNITED STATES OF AMERICA, AS REPRESENTED BY THE SECRETARY, DEPARTMENT OF HEALTH AND HUMAN SERVICES. Application EP. The sequence listing filed with the application follows.

SEQUENCE LISTING (209 sequences)

SEQ ID NO: 1 - protein, 189 aa, Homo sapiens
MTEYKLVVVGADGVGKSALTIQLIQNHFVDEYDPTIEDSYRKQVVIDGETCLLDILDTAGQEEYSAMRDQYMRTGEGFLCVFAINNTKSFEDIHHYREQIKRVKDSEDVPMVLVGNKCDLPSRTVDTKQAQDLARSYGIPFIETSAKTRQRVEDAFYTLVREIRQYRLKKISKEEKTPGCVKIKKCIIM

SEQ ID NO: 2 - protein, 10 aa, Homo sapiens
VVVGADGVGK

SEQ ID NO: 3 - protein, 7 aa, Mus musculus
TIYSNPF

SEQ ID NO: 4 - protein, 7 aa, Mus musculus
SFTDNKR

SEQ ID NO: 5 - protein, 13 aa, Mus musculus
CALRGNAGAKLTF

SEQ ID NO: 6 - protein, 5 aa, Mus musculus
LGHDT

SEQ ID NO: 7 - protein, 6 aa, Mus musculus
YNNKQL

SEQ ID NO: 8 - protein, 15 aa, Mus musculus
CASSSRDWSAETLYF

SEQ ID NO: 9 - protein, 135 aa, Mus musculus
MRPVTCSVLVLLLMLRRSNGDGDSVTQTEGLVTLTEGLPVMLNCTYQTIYSNPFLFWYVQHLNESPRLLLKSFTDNKRTEHQGFHATLHKSSSSFHLQKSSAQLSDSALYYCALRGNAGAKLTFGGGTRLTVRPD

SEQ ID NO: 10 - protein, 134 aa, Mus musculus
MGCRLLSCVAFCLLGIGPLETAVFQTPNYHVTQVGNEVSFNCKQTLGHDTMYWYKQDSKKLLKIMFSYNNKQLIVNETVPRRFSPQSSDKAHLNLRIKSVEPEDSAVYLCASSSRDWSAETLYFGSGTRLTVLE

SEQ ID NO: 11 - protein, 271 aa, Mus musculus
MRPVTCSVLVLLLMLRRSNGDGDSVTQTEGLVTLTEGLPVMLNCTYQTIYSNPFLFWYVQHLNESPRLLLKSFTDNKRTEHQGFHATLHKSSSSFHLQKSSAQLSDSALYYCALRGNAGAKLTFGGGTRLTVRPDIQNPEPAVYQLKDPRSQDSTLCLFTDFDSQINVPKTMESGTFITDKTVLDMKAMDSKSNGAIAWSNQTSFTCQDIFKETNATYPSSDVPCDATLTEKSFETDMNLNFQNLSVMGLRILLLKVAGFNLLMTLRLWSS

SEQ ID NO: 12 - protein, 306 aa, Mus musculus
MGCRLLSCVAFCLLGIGPLETAVFQTPNYHVTQVGNEVSFNCKQTLGHDTMYWYKQDSKKLLKIMFSYNNKQLIVNETVPRRFSPQSSDKAHLNLRIKSVEPEDSAVYLCASSSRDWSAETLYFGSGTRLTVLEDLRNVTPPKVSLFEPSKAEIANKQKATLVCLARGFFPDHVELSWWVNGKEVHSGVSTDPQAYKESNYSYCLSSRLRVSATFWHNPRNHFRCQVQFHGLSEEDKWPEGSPKPVTQNISAEAWGRADCGITSASYHQGVLSATILYEILLGKATLYAVLVSGLVLMAMVKKKNS

SEQ ID NO: 13 - protein, 136 aa, Mus musculus
IQNPEPAVYQLKDPRSQDSTLCLFTDFDSQINVPKTMESGTFITDKTVLDMKAMDSKSNGAIAWSNQTSFTCQDIFKETNATYPSSDVPCDATLTEKSFETDMNLNFQNLSVMGLRILLLKVAGFNLLMTLRLWSS

SEQ ID NO: 14 - protein, 172 aa, Mus musculus
DLRNVTPPKVSLFEPSKAEIANKQKATLVCLARGFFPDHVELSWWVNGKEVHSGVSTDPQAYKESNYSYCLSSRLRVSATFWHNPRNHFRCQVQFHGLSEEDKWPEGSPKPVTQNISAEAWGRADCGITSASYHQGVLSATILYEILLGKATLYAVLVSGLVLMAMVKKKNS

SEQ ID NO: 15 - DNA, 403 bp, Artificial Sequence
  Synthetic
atgcgtcctgtcacctgctcagttcttgtgctcctcctaatgctcaggaggagcaatggcgatggagactccgtgacccagacagaaggcctggtcactctcacagaagggttgcctgtgatgctgaactgcacctatcagactatttactcaaatcctttccttttctggtatgtgcaacatctcaatgaatcccctcggctactcctgaagagcttcacagacaacaagaggaccgagcaccaagggttccacgccactctccataagagcagcagctccttccatctgcagaagtcctcagcgcagctgtcagactctgccctgtactactgtgctctgagggggaatgcaggtgccaagctcacattcggagggggaacaaggttaacggtcagacccg

SEQ ID NO: 16 - DNA, 400 bp, Artificial Sequence
  Synthetic
atgggctgtaggctcctaagctgtgtggccttctgcctcttgggaataggccctttggagacggctgttttccagactccaaactatcatgtcacacaggtgggaaatgaagtgtctttcaattgtaagcaaactctgggccacgatactatgtattggtacaagcaagactctaagaaattgctgaagattatgtttagctacaataataagcaactcattgtaaacgaaacagttccaaggcgcttctcacctcagtcttcagataaagctcatttgaatcttcgaatcaagtctgtagagccggaggactctgctgtgtatctctgtgccagcagctcccgggactggagtgcagaaacgctgtattttggctcaggaaccagactgactgttctcg

SEQ ID NO: 17 - DNA, 816 bp, Artificial Sequence
  Synthetic
atgcgtcctgtcacctgctcagttcttgtgctcctcctaatgctcaggaggagcaatggcgatggagactccgtgacccagacagaaggcctggtcactctcacagaagggttgcctgtgatgctgaactgcacctatcagactatttactcaaatcctttccttttctggtatgtgcaacatctcaatgaatcccctcggctactcctgaagagcttcacagacaacaagaggaccgagcaccaagggttccacgccactctccataagagcagcagctccttccatctgcagaagtcctcagcgcagctgtcagactctgccctgtactactgtgctctgagggggaatgcaggtgccaagctcacattcggagggggaacaaggttaacggtcagacccgacatccagaacccagaacctgctgtgtaccagttaaaagatcctcggtctcaggacagcaccctctgcctgttcaccgactttgactcccaaatcaatgtgccgaaaaccatggaatctggaacgttcatcactgacaaaactgtgctggacatgaaagctatggattccaagagcaatggggccattgcctggagcaaccagacaagcttcacctgccaagatatcttcaaagagaccaacgccacctaccccagttcagacgttccctgtgatgccacgttgactgagaaaagctttgaaacagatatgaacctaaactttcaaaacctgtcagttatgggactccgaatcctcctgctgaaagtagccggatttaacctgctcatgacgctgaggctgtggtccagttga

SEQ ID NO: 18 - DNA, 921 bp, Artificial Sequence
  Synthetic
atgggctgtaggctcctaagctgtgtggccttctgcctcttgggaataggccctttggagacggctgttttccagactccaaactatcatgtcacacaggtgggaaatgaagtgtctttcaattgtaagcaaactctgggccacgatactatgtattggtacaagcaagactctaagaaattgctgaagattatgtttagctacaataataagcaactcattgtaaacgaaacagttccaaggcgcttctcacctcagtcttcagataaagctcatttgaatcttcgaatcaagtctgtagagccggaggactctgctgtgtatctctgtgccagcagctcccgggactggagtgcagaaacgctgtattttggctcaggaaccagactgactgttctcgaggatctgagaaatgtgactccacccaaggtctccttgtttgagccatcaaaagcagagattgcaaacaaacaaaaggctaccctcgtgtgcttggccaggggcttcttccctgaccacgtggagctgagctggtgggtgaatggcaaggaggtccacagtggggtcagcacggaccctcaggcctacaaggagagcaattatagctactgcctgagcagccgcctgagggtctctgctaccttctggcacaatcctcgaaaccacttccgctgccaagtgcagttccatgggctttcagaggaggacaagtggccagagggctcacccaaacctgtcacacagaacatcagtgcagaggcctggggccgagcagactgtggaatcacttcagcatcctatcatcagggggttctgtctgcaaccatcctctatgagatcctactggggaaggccaccctatatgctgtgctggtcagtggcctggtgctgatggccatggtcaagaaaaaaaattcctga

SEQ ID NO: 19 - DNA, 413 bp, Artificial Sequence
  Synthetic
acatccagaacccagaacctgctgtgtaccagttaaaagatcctcggtctcaggacagcaccctctgcctgttcaccgactttgactcccaaatcaatgtgccgaaaaccatggaatctggaacgttcatcactgacaaaactgtgctggacatgaaagctatggattccaagagcaatggggccattgcctggagcaaccagacaagcttcacctgccaagatatcttcaaagagaccaacgccacctaccccagttcagacgttccctgtgatgccacgttgactgagaaaagctttgaaacagatatgaacctaaactttcaaaacctgtcagttatgggactccgaatcctcctgctgaaagtagccggatttaacctgctcatgacgctgaggctgtggtccagttga

SEQ ID NO: 20 - DNA, 521 bp, Artificial Sequence
  Synthetic
aggatctgagaaatgtgactccacccaaggtctccttgtttgagccatcaaaagcagagattgcaaacaaacaaaaggctaccctcgtgtgcttggccaggggcttcttccctgaccacgtggagctgagctggtgggtgaatggcaaggaggtccacagtggggtcagcacggaccctcaggcctacaaggagagcaattatagctactgcctgagcagccgcctgagggtctctgctaccttctggcacaatcctcgaaaccacttccgctgccaagtgcagttccatgggctttcagaggaggacaagtggccagagggctcacccaaacctgtcacacagaacatcagtgcagaggcctggggccgagcagactgtggaatcacttcagcatcctatcatcagggggttctgtctgcaaccatcctctatgagatcctactggggaaggccaccctatatgctgtgctggtcagtggcctagtgctgatggccatggtcaagaaaaaaaattcctga

SEQ ID NO: 21 - DNA, 1815 bp, Artificial Sequence
  Synthetic
atgcgtcctgtcacctgctcagttcttgtgctcctcctaatgctcaggaggagcaatggcgatggagactccgtgacccagacagaaggcctggtcactctcacagaagggttgcctgtgatgctgaactgcacctatcagactatttactcaaatcctttccttttctggtatgtgcaacatctcaatgaatcccctcggctactcctgaagagcttcacagacaacaagaggaccgagcaccaagggttccacgccactctccataagagcagcagctccttccatctgcagaagtcctcagcgcagctgtcagactctgccctgtactactgtgctctgagggggaatgcaggtgccaagctcacattcggagggggaacaaggttaacggtcagacccgacatccagaacccagaacctgctgtgtaccagttaaaagatcctcggtctcaggacagcaccctctgcctgttcaccgactttgactcccaaatcaatgtgccgaaaaccatggaatctggaacgttcatcactgacaaaactgtgctggacatgaaagctatggattccaagagcaatggggccattgcctggagcaaccagacaagcttcacctgccaagatatcttcaaagagaccaacgccacctaccccagttcagacgttccctgtgatgccacgttgactgagaaaagctttgaaacagatatgaacctaaactttcaaaacctgtcagttatgggactccgaatcctcctgctgaaagtagccggatttaacctgctcatgacgctgaggctgtggtccagtcgggccaagcggtccggatccggagccaccaacttcagcctgctgaagcaggccggcgacgtggaggagaaccccggccccatgggctgtaggctcctaagctgtgtggccttctgcctcttgggaataggccctttggagacggctgttttccagactccaaactatcatgtcacacaggtgggaaatgaagtgtctttcaattgtaagcaaactctgggccacgatactatgtattggtacaagcaagactctaagaaattgctgaagattatgtttagctacaataataagcaactcattgtaaacgaaacagttccaaggcgcttctcacctcagtcttcagataaagctcatttgaatcttcgaatcaagtctgtagagccggaggactctgctgtgtatctctgtgccagcagctcccgggactggagtgcagaaacgctgtattttggctcaggaaccagactgactgttctcgaggatctgagaaatgtgactccacccaaggtctccttgtttgagccatcaaaagcagagattgcaaacaaacaaaaggctaccctcgtgtgcttggccaggggcttcttccctgaccacgtggagctgagctggtgggtgaatggcaaggaggtccacagtggggtcagcacggaccctcaggcctacaaggagagcaattatagctactgcctgagcagccgcctgagggtctctgctaccttctggcacaatcctcgaaaccacttccgctgccaagtgcagttccatgggctttcagaggaggacaagtggccagagggctcacccaaacctgtcacacagaacatcagtgcagaggcctggggccgagcagactgtggaatcacttcagcatcctatcatcagggggttctgtctgcaaccatcctctatgagatcctactggggaaggccaccctatatgctgtgctggtcagtggcctggtgctgatggccatggtcaagaaaaaaaattcctga

SEQ ID NO: 22 - DNA, 21 bp, Artificial Sequence
  Synthetic
actatttactcaaatcctttc

SEQ ID NO: 23 - DNA, 21 bp, Artificial Sequence
  Synthetic
agcttcacagacaacaagagg

SEQ ID NO: 24 - DNA, 33 bp, Artificial Sequence
  Synthetic
gctctgagggggaatgcaggtgccaagctcaca

SEQ ID NO: 25 - DNA, 15 bp, Artificial Sequence
  Synthetic
ctgggccacgatact

SEQ ID NO: 26 - DNA, 18 bp, Artificial Sequence
  Synthetic
tacaataataagcaactc

SEQ ID NO: 27 - DNA, 39 bp, Artificial Sequence
  Synthetic
gccagcagctcccgggactggagtgcagaaacgctgtat

SEQ ID NO: 28 - protein, 27 aa, Artificial Sequence
  Synthetic
RAKRSGSGATNFSLLKQAGDVEENPGP

SEQ ID NO: 29 - protein, 189 aa, Homo sapiens [sequence omitted]

SEQ ID NO: 30 - protein, 10 aa, Homo sapiens
VVVGAGGVGK

SEQ ID NO: 31 - protein, 9 aa, Homo sapiens
VVGAGGVGK

SEQ ID NO: 32 - protein, 189 aa, Homo sapiens
MTEYKLVVVGAVGVGKSALTIQLIQNHFVDEYDPTIEDSYRKQVVIDGETCLLDILDTAGQEEYSAMRDQYMRTGEGFLCVFAINNTKSFEDIHHYREQIKRVKDSEDVPMVLVGNKCDLPSRTVDTKQAQDLARSYGIPFIETSAKTRQRVEDAFYTLVREIRQYRLKKISKEEKTPGCVKIKKCIIM

SEQ ID NO: 33 - protein, 10 aa, Homo sapiens
VVVGAVGVGK

SEQ ID NO: 34 - protein, 9 aa, Homo sapiens
VVGADGVGK

SEQ ID NO: 35 - protein, 9 aa, Homo sapiens
VVGAVGVGK

SEQ ID NO: 36 - protein, 9 aa, Homo sapiens
VVGACGVGK

SEQ ID NO: 37 - protein, 10 aa, Homo sapiens
VVVGACGVGK

SEQ ID NO: 38 - protein, 9 aa, Homo sapiens
VVGARGVGK

SEQ ID NO: 39 - protein, 10 aa, Homo sapiens
VVVGARGVGK

SEQ ID NO: 40 - protein, 16 aa, Mus musculus
CAMREDTGANTGKLTF

SEQ ID NO: 41 - protein, 15 aa, Mus musculus
CASSQDSLGRAEQFF

SEQ ID NO: 42 - protein, 15 aa, Mus musculus
CASSSDWGGAETLYF

SEQ ID NO: 43 - protein, 16 aa, Mus musculus
CASSSGLGSSAETLYF

SEQ ID NO: 44 - DNA, 81 bp, Artificial Sequence
  Synthetic
cgggccaagcggtccggatccggagccaccaacttcagcctgctgaagcaggccggcgacgtggaggagaaccccggcccc

SEQ ID NO: 45 - protein, 604 aa, Artificial Sequence
  Synthetic
MRPVTCSVLVLLLMLRRSNGDGDSVTQTEGLVTLTEGLPVMLNCTYQTIYSNPFLFWYVQHLNESPRLLLKSFTDNKRTEHQGFHATLHKSSSSFHLQKSSAQLSDSALYYCALRGNAGAKLTFGGGTRLTVRPDIQNPEPAVYQLKDPRSQDSTLCLFTDFDSQINVPKTMESGTFITDKTVLDMKAMDSKSNGAIAWSNQTSFTCQDIFKETNATYPSSDVPCDATLTEKSFETDMNLNFQNLSVMGLRILLLKVAGFNLLMTLRLWSSRAKRSGSGATNFSLLKQAGDVEENPGPMGCRLLSCVAFCLLGIGPLETAVFQTPNYHVTQVGNEVSFNCKQTLGHDTMYWYKQDSKKLLKIMFSYNNKQLIVNETVPRRFSPQSSDKAHLNLRIKSVEPEDSAVYLCASSSRDWSAETLYFGSGTRLTVLEDLRNVTPPKVSLFEPSKAEIANKQKATLVCLARGFFPDHVELSWWVNGKEVHSGVSTDPQAYKESNYSYCLSSRLRVSATFWHNPRNHFRCQVQFHGLSEEDKWPEGSPKPVTQNISAEAWGRADCGITSASYHQGVLSATILYEILLGKATLYAVLVSGLVLMAMVKKKNS

SEQ ID NO: 46 - protein, 13 aa, Artificial Sequence
  Synthetic
  MISC_FEATURE (2)..(2): Xaa is Arg, Asn, Asp, Cys, Glu, Gln, Gly, His, Ile, Leu, Lys, Met, Phe, Pro, Ser, Thr, Trp, Tyr, or Val.
CXLRGNAGAKLTF

SEQ ID NO: 47 - protein, 13 aa, Artificial Sequence
  Synthetic
  MISC_FEATURE (3)..(3): Xaa is Ala, Arg, Asn, Asp, Cys, Glu, Gln, Gly, His, Ile, Lys, Met, Phe, Pro, Ser, Thr, Trp, Tyr, or Val.
CAXRGNAGAKLTF

SEQ ID NO: 48 - protein, 13 aa, Artificial Sequence
  Synthetic
  MISC_FEATURE (4)..(4): Xaa is Ala, Asn, Asp, Cys, Glu, Gln, Gly, His, Ile, Leu, Lys, Met, Phe, Pro, Ser, Thr, Trp, Tyr, or Val.
CALXGNAGAKLTF

SEQ ID NO: 49 - protein, 13 aa, Artificial Sequence
  Synthetic
  MISC_FEATURE (5)..(5): Xaa is Ala, Arg, Asn, Asp, Cys, Glu, Gln, His, Ile, Leu, Lys, Met, Phe, Pro, Ser, Thr, Trp, Tyr, or Val.
CALRXNAGAKLTF

SEQ ID NO: 50 - protein, 13 aa, Artificial Sequence
  Synthetic
  MISC_FEATURE (6)..(6): Xaa is Ala, Arg, Asp, Cys, Glu, Gln, Gly, His, Ile, Leu, Lys, Met, Phe, Pro, Ser, Thr, Trp, Tyr, or Val.
CALRGXAGAKLTF

SEQ ID NO: 51 - protein, 13 aa, Artificial Sequence
  Synthetic
  MISC_FEATURE (7)..(7): Xaa is Arg, Asn, Asp, Cys, Glu, Gln, Gly, His, Ile, Leu, Lys, Met, Phe, Pro, Ser, Thr, Trp, Tyr, or Val.
CALRGNXGAKLTF

SEQ ID NO: 52 - protein, 13 aa, Artificial Sequence
  Synthetic
  MISC_FEATURE (8)..(8): Xaa is Ala, Arg, Asn, Asp, Cys, Glu, Gln, His, Ile, Leu, Lys, Met, Phe, Pro, Ser, Thr, Trp, Tyr, or Val.
CALRGNAXAKLTF

SEQ ID NO: 53 - protein, 13 aa, Artificial Sequence
  Synthetic
  MISC_FEATURE (9)..(9): Xaa is Arg, Asn, Asp, Cys, Glu, Gln, Gly, His, Ile, Leu, Lys, Met, Phe, Pro, Ser, Thr, Trp, Tyr, or Val.
CALRGNAGXKLTF

SEQ ID NO: 54 - protein, 13 aa, Artificial Sequence
  Synthetic
  MISC_FEATURE (10)..(10): Xaa is Ala, Arg, Asn, Asp, Cys, Glu, Gln, Gly, His, Ile, Leu, Met, Phe, Pro, Ser, Thr, Trp, Tyr, or Val.
CALRGNAGAXLTF

SEQ ID NO: 55 - protein, 13 aa, Artificial Sequence
  Synthetic
  MISC_FEATURE (11)..(11): Xaa is Ala, Arg, Asn, Asp, Cys, Glu, Gln, Gly, His, Ile, Lys, Met, Phe, Pro, Ser, Thr, Trp, Tyr, or Val.
CALRGNAGAKXTF

SEQ ID NO: 56 - protein, 13 aa, Artificial Sequence
  Synthetic
  MISC_FEATURE (12)..(12): Xaa is Ala, Arg, Asn, Asp, Cys, Glu, Gln, Gly, His, Ile, Leu, Lys, Met, Phe, Pro, Ser, Trp, Tyr, or Val.
CALRGNAGAKLXF

SEQ ID NO: 57 - protein, 15 aa, Artificial Sequence
  Synthetic
  MISC_FEATURE (2)..(2): Xaa is Arg, Asn, Asp, Cys, Glu, Gln, Gly, His, Ile, Leu, Lys, Met, Phe, Pro, Ser, Thr, Trp, Tyr, or Val.
CXSSSRDWSAETLYF

SEQ ID NO: 58 - protein, 15 aa, Artificial Sequence
  Synthetic
  MISC_FEATURE (3)..(3): Xaa is Ala, Arg, Asn, Asp, Cys, Glu, Gln, Gly, His, Ile, Leu, Lys, Met, Phe, Pro, Thr, Trp, Tyr, or Val.
CAXSSRDWSAETLYF

SEQ ID NO: 59 - protein, 15 aa, Artificial Sequence
  Synthetic
  MISC_FEATURE (4)..(4): Xaa is Ala, Arg, Asn, Asp, Cys, Glu, Gln, Gly, His, Ile, Leu, Lys, Met, Phe, Pro, Thr, Trp, Tyr, or Val.
CASXSRDWSAETLYF

SEQ ID NO: 60 - protein, 15 aa, Artificial Sequence
  Synthetic
  MISC_FEATURE (5)..(5): Xaa is Ala, Arg, Asn, Asp, Cys, Glu, Gln, Gly, His, Ile, Leu, Lys, Met, Phe, Pro, Thr, Trp, Tyr, or Val.
CASSXRDWSAETLYF

SEQ ID NO: 61 - protein, 15 aa, Artificial Sequence
  Synthetic
  MISC_FEATURE (6)..(6): Xaa is Ala, Asn, Asp, Cys, Glu, Gln, Gly, His, Ile, Leu, Lys, Met, Phe, Pro, Ser, Thr, Trp, Tyr, or Val,
CASSSXDWSAETLYF

SEQ ID NO: 62 - protein, 15 aa, Artificial Sequence
  Synthetic
  MISC_FEATURE (7)..(7): Xaa is Ala, Arg, Asn, Cys, Glu, Gln, Gly, His, Ile, Leu, Lys, Met, Phe, Pro, Ser, Thr, Trp, Tyr, or Val.
CASSSRXWSAETLYF

SEQ ID NO: 63 - protein, 15 aa, Artificial Sequence
  Synthetic
  MISC_FEATURE (8)..(8): Xaa is Ala, Arg, Asn, Asp, Cys, Glu, Gln, Gly, His, Ile, Leu, Lys, Met, Phe, Pro, Ser, Thr, Tyr, or Val.
CASSSRDXSAETLYF

SEQ ID NO: 64 - protein, 15 aa, Artificial Sequence
  Synthetic
  MISC_FEATURE (9)..(9): Xaa is Ala, Arg, Asn, Asp, Cys, Glu, Gln, Gly, His, Ile, Leu, Lys, Met, Phe, Pro, Thr, Trp, Tyr, or Val.
CASSSRDWXAETLYF

SEQ ID NO: 65 - protein, 15 aa, Artificial Sequence
  Synthetic
  MISC_FEATURE (10)..(10): Xaa is Arg, Asn, Asp, Cys, Glu, Gln, Gly, His, Ile, Leu, Lys, Met, Phe, Pro, Ser, Thr, Trp, Tyr, or Val.
CASSSRDWSXETLYF

SEQ ID NO: 66 - protein, 15 aa, Artificial Sequence
  Synthetic
  MISC_FEATURE (11)..(11): Xaa is Ala, Arg, Asn, Asp, Cys, Gln, Gly, His, Ile, Leu, Lys, Met, Phe, Pro, Ser, Thr, Trp, Tyr, or Val.
CASSSRDWSAXTLYF

SEQ ID NO: 67 - protein, 15 aa, Artificial Sequence
  Synthetic
  MISC_FEATURE (12)..(12): Xaa is Ala, Arg, Asn, Asp, Cys, Glu, Gln, Gly, His, Ile, Leu, Lys, Met, Phe, Pro, Ser, Trp, Tyr, or Val.
CASSSRDWSAEXLYF

SEQ ID NO: 68 - protein, 15 aa, Artificial Sequence
  Synthetic
  MISC_FEATURE (13)..(13): Xaa is Ala, Arg, Asn, Asp, Cys, Glu, Gln, Gly, His, Ile, Lys, Met, Phe, Pro, Ser, Thr, Trp, Tyr, or Val.
CASSSRDWSAETXYF

SEQ ID NO: 69 - protein, 15 aa, Artificial Sequence
  Synthetic
  MISC_FEATURE (14)..(14): Xaa is Ala, Arg, Asn, Asp, Cys, Glu, Gln, Gly, His, Ile, Leu, Lys, Met, Phe, Pro, Ser, Thr, Trp, or Val.
CASSSRDWSAETLXF

SEQ ID NO: 70 - protein, 135 aa, Artificial Sequence
  Synthetic
  MISC_FEATURE (113)..(113): Xaa is Arg, Asn, Asp, Cys, Glu, Gln, Gly, His, Ile, Leu, Lys, Met, Phe, Pro, Ser, Thr, Trp, Tyr, or Val.
MRPVTCSVLVLLLMLRRSNGDGDSVTQTEGLVTLTEGLPVMLNCTYQTIYSNPFLFWYVQHLNESPRLLLKSFTDNKRTEHQGFHATLHKSSSSFHLQKSSAQLSDSALYYCXLRGNAGAKLTFGGGTRLTVRPD

SEQ ID NO: 71 - protein, 135 aa, Artificial Sequence
  Synthetic
  MISC_FEATURE (114)..(114): Xaa is Ala, Arg, Asn, Asp, Cys, Glu, Gln, Gly, His, Ile, Lys, Met, Phe, Pro, Ser, Thr, Trp, Tyr, or val.
MRPVTCSVLVLLLMLRRSNGDGDSVTQTEGLVTLTEGLPVMLNCTYQTIYSNPFLFWYVQHLNESPRLLLKSFTDNKRTEHQGFHATLHKSSSSFHLQKSSAQLSDSALYYCAXRGNAGAKLTFGGGTRLTVRPD

SEQ ID NO: 72 - protein, 135 aa, Artificial Sequence
  Synthetic
  MISC_FEATURE (115)..(115): Xaa is Ala, Asn, Asp, Cys, Glu, Gln, Gly, His, Ile, Leu, Lys, Met, Phe, Pro, Ser, Thr, Trp, Tyr, or Val.
MRPVTCSVLVLLLMLRRSNGDGDSVTQTEGLVTLTEGLPVMLNCTYQTIYSNPFLFWYVQHLNESPRLLLKSFTDNKRTEHQGFHATLHKSSSSFHLQKSSAQLSDSALYYCALXGNAGAKLTFGGGTRLTVRPD

SEQ ID NO: 73 - protein, 135 aa, Artificial Sequence
  Synthetic
  MISC_FEATURE (116)..(116): Xaa is Ala, Arg, Asn, Asp, Cys, Glu, Gln, His, Ile, Leu, Lys, Met, Phe, Pro, Ser, Thr, Trp, Tyr, or Val.
MRPVTCSVLVLLLMLRRSNGDGDSVTQTEGLVTLTEGLPVMLNCTYQTIYSNPFLFWYVQHLNESPRLLLKSFTDNKRTEHQGFHATLHKSSSSFHLQKSSAQLSDSALYYCALRXNAGAKLTFGGGTRLTVRPD

SEQ ID NO: 74 - protein, 135 aa, Artificial Sequence
  Synthetic
  MISC_FEATURE (117)..(117): Xaa is Ala, Arg, Asp, Cys, Glu, Gln, Gly, His, Ile, Leu, Lys, Met, Phe, Pro, Ser, Thr, Trp, Tyr, or Val.
MRPVTCSVLVLLLMLRRSNGDGDSVTQTEGLVTLTEGLPVMLNCTYQTIYSNPFLFWYVQHLNESPRLLLKSFTDNKRTEHQGFHATLHKSSSSFHLQKSSAQLSDSALYYCALRGXAGAKLTFGGGTRLTVRPD

SEQ ID NO: 75 - protein, 135 aa, Artificial Sequence
  Synthetic
  MISC_FEATURE (118)..(118): Xaa is Arg, Asn, Asp, Cys, Glu, Gln, Gly, His, Ile, Leu, Lys, Met, Phe, Pro, Ser, Thr, Trp, Tyr, or Val.
MRPVTCSVLVLLLMLRRSNGDGDSVTQTEGLVTLTEGLPVMLNCTYQTIYSNPFLFWYVQHLNESPRLLLKSFTDNKRTEHQGFHATLHKSSSSFHLQKSSAQLSDSALYYCALRGNXGAKLTFGGGTRLTVRPD

SEQ ID NO: 76 - protein, 135 aa, Artificial Sequence
  Synthetic
  MISC_FEATURE (119)..(119): Xaa is Ala, Arg, Asn, Asp, Cys, Glu, Gln, His, Ile, Leu, Lys, Met, Phe, Pro, Ser, Thr, Trp, Tyr, or Val.
MRPVTCSVLVLLLMLRRSNGDGDSVTQTEGLVTLTEGLPVMLNCTYQTIYSNPFLFWYVQHLNESPRLLLKSFTDNKRTEHQGFHATLHKSSSSFHLQKSSAQLSDSALYYCALRGNAXAKLTFGGGTRLTVRPD

SEQ ID NO: 77 - protein, 135 aa, Artificial Sequence
  Synthetic
  MISC_FEATURE (120)..(120): Xaa is Arg, Asn, Asp, Cys, Glu, Gln, Gly, His, Ile, Leu, Lys, Met, Phe, Pro, Ser, Thr, Trp, Tyr, or Val.
MRPVTCSVLVLLLMLRRSNGDGDSVTQTEGLVTLTEGLPVMLNCTYQTIYSNPFLFWYVQHLNESPRLLLKSFTDNKRTEHQGFHATLHKSSSSFHLQKSSAQLSDSALYYCALRGNAGXKLTFGGGTRLTVRPD

SEQ ID NO: 78 - protein, 135 aa, Artificial Sequence
  Synthetic
  MISC_FEATURE (121)..(121): Xaa is Ala, Arg, Asn, Asp, Cys, Glu, Gln, Gly, His, Ile, Leu, Met, Phe, Pro, Ser, Thr, Trp, Tyr, or val.
MRPVTCSVLVLLLMLRRSNGDGDSVTQTEGLVTLTEGLPVMLNCTYQTIYSNPFLFWYVQHLNESPRLLLKSFTDNKRTEHQGFHATLHKSSSSFHLQKSSAQLSDSALYYCALRGNAGAXLTFGGGTRLTVRPD

SEQ ID NO: 79 - protein, 135 aa, Artificial Sequence
  Synthetic
  MISC_FEATURE (122)..(122): Xaa is Ala, Arg, Asn, Asp, Cys, Glu, Gln, Gly, His, Ile, Lys, Met, Phe, Pro, Ser, Thr, Trp, Tyr, or Val.
MRPVTCSVLVLLLMLRRSNGDGDSVTQTEGLVTLTEGLPVMLNCTYQTIYSNPFLFWYVQHLNESPRLLLKSFTDNKRTEHQGFHATLHKSSSSFHLQKSSAQLSDSALYYCALRGNAGAKXTFGGGTRLTVRPD

SEQ ID NO: 80 - protein, 135 aa, Artificial Sequence
  Synthetic
  MISC_FEATURE (123)..(123): Xaa is Ala, Arg, Asn, Asp, Cys, Glu, Gln, Gly, His, Ile, Leu, Lys, Met, Phe, Pro, Ser, Trp, Tyr, or Val.
MRPVTCSVLVLLLMLRRSNGDGDSVTQTEGLVTLTEGLPVMLNCTYQTIYSNPFLFWYVQHLNESPRLLLKSFTDNKRTEHQGFHATLHKSSSSFHLQKSSAQLSDSALYYCALRGNAGAKLXFGGGTRLTVRPD

SEQ ID NO: 81 - protein, 134 aa, Artificial Sequence
  Synthetic
  MISC_FEATURE (111)..(111): Xaa is Arg, Asn, Asp, Cys, Glu, Gln, Gly, His, Ile, Leu, Lys, Met, Phe, Pro, Ser, Thr, Trp, Tyr, or Val.
MGCRLLSCVAFCLLGIGPLETAVFQTPNYHVTQVGNEVSFNCKQTLGHDTMYWYKQDSKKLLKIMFSYNNKQLIVNETVPRRFSPQSSDKAHLNLRIKSVEPEDSAVYLCXSSSRDWSAETLYFGSGTRLTVLE

SEQ ID NO: 82 - protein, 134 aa, Artificial Sequence
  Synthetic
  MISC_FEATURE (112)..(112): Xaa is Ala, Arg, Asn, Asp, Cys, Glu, Gln, Gly, His, Ile, Leu, Lys, Met, Phe, Pro, Thr, Trp, Tyr, or Val.
MGCRLLSCVAFCLLGIGPLETAVFQTPNYHVTQVGNEVSFNCKQTLGHDTMYWYKQDSKKLLKIMFSYNNKQLIVNETVPRRFSPQSSDKAHLNLRIKSVEPEDSAVYLCAXSSRDWSAETLYFGSGTRLTVLE

SEQ ID NO: 83 - protein, 134 aa, Artificial Sequence
  Synthetic
  MISC_FEATURE (113)..(113): X is Ala, Arg, Asn, Asp, Cys, Glu, Gln, Gly, His, Ile, Leu, Lys, Met, Phe, Pro, Thr, Trp, Tyr, or Val.
MGCRLLSCVAFCLLGIGPLETAVFQTPNYHVTQVGNEVSFNCKQTLGHDTMYWYKQDSKKLLKIMFSYNNKQLIVNETVPRRFSPQSSDKAHLNLRIKSVEPEDSAVYLCASXSRDWSAETLYFGSGTRLTVLE

SEQ ID NO: 84 - protein, 134 aa, Artificial Sequence
  Synthetic
  MISC_FEATURE (114)..(114): Xaa is Ala, Arg, Asn, Asp, Cys, Glu, Gln, Gly, His, Ile, Leu, Lys, Met, Phe, Pro, Thr, Trp, Tyr, or Val.
MGCRLLSCVAFCLLGIGPLETAVFQTPNYHVTQVGNEVSFNCKQTLGHDTMYWYKQDSKKLLKIMFSYNNKQLIVNETVPRRFSPQSSDKAHLNLRIKSVEPEDSAVYLCASSXRDWSAETLYFGSGTRLTVLE

SEQ ID NO: 85 - protein, 134 aa, Artificial Sequence
  Synthetic
  MISC_FEATURE (115)..(115): Xaa is Ala, Asn, Asp, Cys, Glu, Gln, Gly, His, Ile, Leu, Lys, Met, Phe, Pro, Ser, Thr, Trp, Tyr, or Val.
MGCRLLSCVAFCLLGIGPLETAVFQTPNYHVTQVGNEVSFNCKQTLGHDTMYWYKQDSKKLLKIMFSYNNKQLIVNETVPRRFSPQSSDKAHLNLRIKSVEPEDSAVYLCASSSXDWSAETLYFGSGTRLTVLE

SEQ ID NO: 86 - protein, 134 aa, Artificial Sequence
  Synthetic
  MISC_FEATURE (116)..(116): Xaa is Ala, Arg, Asn, Cys, Glu, Gln, Gly, His, Ile, Leu, Lys, Met, Phe, Pro, Ser, Thr, Trp, Tyr, or Val.
MGCRLLSCVAFCLLGIGPLETAVFQTPNYHVTQVGNEVSFNCKQTLGHDTMYWYKQDSKKLLKIMFSYNNKQLIVNETVPRRFSPQSSDKAHLNLRIKSVEPEDSAVYLCASSSRXWSAETLYFGSGTRLTVLE

SEQ ID NO: 87 - protein, 134 aa, Artificial Sequence
  Synthetic
  MISC_FEATURE (117)..(117): Xaa is Ala, Arg, Asn, Asp, Cys, Glu, Gln, Gly, His, Ile, Leu, Lys, Met, Phe, Pro, Ser, Thr, Tyr, or Val.
MGCRLLSCVAFCLLGIGPLETAVFQTPNYHVTQVGNEVSFNCKQTLGHDTMYWYKQDSKKLLKIMFSYNNKQLIVNETVPRRFSPQSSDKAHLNLRIKSVEPEDSAVYLCASSSRDXSAETLYFGSGTRLTVLE

SEQ ID NO: 88 - protein, 134 aa, Artificial Sequence
  Synthetic
  MISC_FEATURE (118)..(118): Xaa is Ala, Arg, Asn, Asp, Cys, Glu, Gln, Gly, His, Ile, Leu, Lys, Met, Phe, Pro, Thr, Trp, Tyr, or Val.
MGCRLLSCVAFCLLGIGPLETAVFQTPNYHVTQVGNEVSFNCKQTLGHDTMYWYKQDSKKLLKIMFSYNNKQLIVNETVPRRFSPQSSDKAHLNLRIKSVEPEDSAVYLCASSSRDWXAETLYFGSGTRLTVLE

SEQ ID NO: 89 - protein, 134 aa, Artificial Sequence
  Synthetic
  MISC_FEATURE (119)..(119): Xaa is Arg, Asn, Asp, Cys, Glu, Gln, Gly, His, Ile, Leu, Lys, Met, Phe, Pro, Ser, Thr, Trp, Tyr, or Val.
MGCRLLSCVAFCLLGIGPLETAVFQTPNYHVTQVGNEVSFNCKQTLGHDTMYWYKQDSKKLLKIMFSYNNKQLIVNETVPRRFSPQSSDKAHLNLRIKSVEPEDSAVYLCASSSRDWSXETLYFGSGTRLTVLE

SEQ ID NO: 90 - protein, 134 aa, Artificial Sequence
  Synthetic
  MISC_FEATURE (120)..(120): Xaa is Ala, Arg, Asn, Asp, Cys, Gln, Gly, His, Ile, Leu, Lys, Met, Phe, Pro, Ser, Thr, Trp, Tyr, or Val.
MGCRLLSCVAFCLLGIGPLETAVFQTPNYHVTQVGNEVSFNCKQTLGHDTMYWYKQDSKKLLKIMFSYNNKQLIVNETVPRRFSPQSSDKAHLNLRIKSVEPEDSAVYLCASSSRDWSAXTLYFGSGTRLTVLE

SEQ ID NO: 91 - protein, 134 aa, Artificial Sequence
  Synthetic
  MISC_FEATURE (121)..(121): Xaa is Ala, Arg, Asn, Asp, Cys, Glu, Gln, Gly, His, Ile, Leu, Lys, Met, Phe, Pro, Ser, Trp, Tyr, or Val.
MGCRLLSCVAFCLLGIGPLETAVFQTPNYHVTQVGNEVSFNCKQTLGHDTMYWYKQDSKKLLKIMFSYNNKQLIVNETVPRRFSPQSSDKAHLNLRIKSVEPEDSAVYLCASSSRDWSAEXLYFGSGTRLTVLE

SEQ ID NO: 92 - protein, 134 aa, Artificial Sequence
  Synthetic
  MISC_FEATURE (122)..(122): Xaa is Ala, Arg, Asn, Asp, Cys, Glu, Gln, Gly, His, Ile, Lys, Met, Phe, Pro, Ser, Thr, Trp, Tyr, or Val.
MGCRLLSCVAFCLLGIGPLETAVFQTPNYHVTQVGNEVSFNCKQTLGHDTMYWYKQDSKKLLKIMFSYNNKQLIVNETVPRRFSPQSSDKAHLNLRIKSVEPEDSAVYLCASSSRDWSAETXYFGSGTRLTVLE

SEQ ID NO: 93 - protein, 134 aa, Artificial Sequence
  'Synthetic
  MISC_FEATURE (123)..(123): Xaa is Ala, Arg, Asn, Asp, Cys, Glu, Gln, Gly, His, Ile, Leu, Lys, Met, Phe, Pro, Ser, Thr, Trp, or Val.
MGCRLLSCVAFCLLGIGPLETAVFQTPNYHVTQVGNEVSFNCKQTLGHDTMYWYKQDSKKLLKIMFSYNNKQLIVNETVPRRFSPQSSDKAHLNLRIKSVEPEDSAVYLCASSSRDWSAETLXFGSGTRLTVLE

SEQ ID NO: 94 - protein, 271 aa, Artificial Sequence
  Synthetic
  MISC_FEATURE (113)..(113): Xaa is Arg, Asn, Asp, Cys, Glu, Gln, Gly, His, Ile, Leu, Lys, Met, Phe, Pro, Ser, Thr, Trp, Tyr, or Val.
MRPVTCSVLVLLLMLRRSNGDGDSVTQTEGLVTLTEGLPVMLNCTYQTIYSNPFLFWYVQHLNESPRLLLKSFTDNKRTEHQGFHATLHKSSSSFHLQKSSAQLSDSALYYCXLRGNAGAKLTFGGGTRLTVRPDIQNPEPAVYQLKDPRSQDSTLCLFTDFDSQINVPKTMESGTFITDKTVLDMKAMDSKSNGAIAWSNQTSFTCQDIFKETNATYPSSDVPCDATLTEKSFETDMNLNFQNLSVMGLRILLLKVAGFNLLMTLRLWSS

SEQ ID NO: 95 - protein, 271 aa, Artificial Sequence
  Synthetic
  MISC_FEATURE (114)..(114): Xaa is Ala, Arg, Asn, Asp, Cys, Glu, Gln, Gly, His, Ile, Lys, Met, Phe, Pro, Ser, Thr, Trp, Tyr, or Val.
MRPVTCSVLVLLLMLRRSNGDGDSVTQTEGLVTLTEGLPVMLNCTYQTIYSNPFLFWYVQHLNESPRLLLKSFTDNKRTEHQGFHATLHKSSSSFHLQKSSAQLSDSALYYCAXRGNAGAKLTFGGGTRLTVRPDIQNPEPAVYQLKDPRSQDSTLCLFTDFDSQINVPKTMESGTFITDKTVLDMKAMDSKSNGAIAWSNQTSFTCQDIFKETNATYPSSDVPCDATLTEKSFETDMNLNFQNLSVMGLRILLLKVAGFNLLMTLRLWSS

SEQ ID NO: 96 - protein, 271 aa, Artificial Sequence
  Synthetic
  MISC_FEATURE (115)..(115): Xaa is Ala, Asn, Asp, Cys, Glu, Gln, Gly, His, Ile, Leu, Lys, Met, Phe, Pro, Ser, Thr, Trp, Tyr, or Val.
MRPVTCSVLVLLLMLRRSNGDGDSVTQTEGLVTLTEGLPVMLNCTYQTIYSNPFLFWYVQHLNESPRLLLKSFTDNKRTEHQGFHATLHKSSSSFHLQKSSAQLSDSALYYCALXGNAGAKLTFGGGTRLTVRPDIQNPEPAVYQLKDPRSQDSTLCLFTDFDSQINVPKTMESGTFITDKTVLDMKAMDSKSNGAIAWSNQTSFTCQDIFKETNATYPSSDVPCDATLTEKSFETDMNLNFQNLSVMGLRILLLKVAGFNLLMTLRLWSS

SEQ ID NO: 97 - protein, 271 aa, Artificial Sequence
  Synthetic
  MISC_FEATURE (116)..(116): Xaa is Ala, Arg, Asn, Asp, Cys, Glu, Gln, His, Ile, Leu, Lys, Met, Phe, Pro, Ser, Thr, Trp, Tyr, or Val.
MRPVTCSVLVLLLMLRRSNGDGDSVTQTEGLVTLTEGLPVMLNCTYQTIYSNPFLFWYVQHLNESPRLLLKSFTDNKRTEHQGFHATLHKSSSSFHLQKSSAQLSDSALYYCALRXNAGAKLTFGGGTRLTVRPDIQNPEPAVYQLKDPRSQDSTLCLFTDFDSQINVPKTMESGTFITDKTVLDMKAMDSKSNGAIAWSNQTSFTCQDIFKETNATYPSSDVPCDATLTEKSFETDMNLNFQNLSVMGLRILLLKVAGFNLLMTLRLWSS

SEQ ID NO: 98 - protein, 271 aa, Artificial Sequence
  Synthetic
  MISC_FEATURE (117)..(117): Xaa is Ala, Arg, Asp, Cys, Glu, Gln, Gly, His, Ile, Leu, Lys, Met, Phe, Pro, Ser, Thr, Trp, Tyr, or Val.
MRPVTCSVLVLLLMLRRSNGDGDSVTQTEGLVTLTEGLPVMLNCTYQTIYSNPFLFWYVQHLNESPRLLLKSFTDNKRTEHQGFHATLHKSSSSFHLQKSSAQLSDSALYYCALRGXAGAKLTFGGGTRLTVRPDIQNPEPAVYQLKDPRSQDSTLCLFTDFDSQINVPKTMESGTFITDKTVLDMKAMDSKSNGAIAWSNQTSFTCQDIFKETNATYPSSDVPCDATLTEKSFETDMNLNFQNLSVMGLRILLLKVAGFNLLMTLRLWSS

SEQ ID NO: 99 - protein, 271 aa, Artificial Sequence
  Synthetic
  MISC_FEATURE (118)..(118): Xaa is Arg, Asn, Asp, Cys, Glu, Gln, Gly, His, Ile, Leu, Lys, Met, Phe, Pro, Ser, Thr, Trp, Tyr, or Val.
MRPVTCSVLVLLLMLRRSNGDGDSVTQTEGLVTLTEGLPVMLNCTYQTIYSNPFLFWYVQHLNESPRLLLKSFTDNKRTEHQGFHATLHKSSSSFHLQKSSAQLSDSALYYCALRGNXGAKLTFGGGTRLTVRPDIQNPEPAVYQLKDPRSQDSTLCLFTDFDSQINVPKTMESGTFITDKTVLDMKAMDSKSNGAIAWSNQTSFTCQDIFKETNATYPSSDVPCDATLTEKSFETDMNLNFQNLSVMGLRILLLKVAGFNLLMTLRLWSS

SEQ ID NO: 100 - protein, 271 aa, Artificial Sequence
  Synthetic
  MISC_FEATURE (119)..(119): Xaa is Ala, Arg, Asn, Asp, Cys, Glu, Gln, His, Ile, Leu, Lys, Met, Phe, Pro, Ser, Thr, Trp, Tyr, or Val.
MRPVTCSVLVLLLMLRRSNGDGDSVTQTEGLVTLTEGLPVMLNCTYQTIYSNPFLFWYVQHLNESPRLLLKSFTDNKRTEHQGFHATLHKSSSSFHLQKSSAQLSDSALYYCALRGNAXAKLTFGGGTRLTVRPDIQNPEPAVYQLKDPRSQDSTLCLFTDFDSQINVPKTMESGTFITDKTVLDMKAMDSKSNGAIAWSNQTSFTCQDIFKETNATYPSSDVPCDATLTEKSFETDMNLNFQNLSVMGLRILLLKVAGFNLLMTLRLWSS

SEQ ID NO: 101 - protein, 271 aa, Artificial Sequence
  Synthetic
  MISC_FEATURE (120)..(120): Xaa is Arg, Asn, Asp, Cys, Glu, Gln, Gly, His, Ile, Leu, Lys, Met, Phe, Pro, Ser, Thr, Trp, Tyr, or Val.
MRPVTCSVLVLLLMLRRSNGDGDSVTQTEGLVTLTEGLPVMLNCTYQTIYSNPFLFWYVQHLNESPRLLLKSFTDNKRTEHQGFHATLHKSSSSFHLQKSSAQLSDSALYYCALRGNAGXKLTFGGGTRLTVRPDIQNPEPAVYQLKDPRSQDSTLCLFTDFDSQINVPKTMESGTFITDKTVLDMKAMDSKSNGAIAWSNQTSFTCQDIFKETNATYPSSDVPCDATLTEKSFETDMNLNFQNLSVMGLRILLLKVAGFNLLMTLRLWSS

SEQ ID NO: 102 - protein, 271 aa, Artificial Sequence
  Synthetic
  MISC_FEATURE (121)..(121): Xaa is Ala, Arg, Asn, Asp, Cys, Glu, Gln, Gly, His, Ile, Leu, Met, Phe, Pro, Ser, Thr, Trp, Tyr, or Val.
MRPVTCSVLVLLLMLRRSNGDGDSVTQTEGLVTLTEGLPVMLNCTYQTIYSNPFLFWYVQHLNESPRLLLKSFTDNKRTEHQGFHATLHKSSSSFHLQKSSAQLSDSALYYCALRGNAGAXLTFGGGTRLTVRPDIQNPEPAVYQLKDPRSQDSTLCLFTDFDSQINVPKTMESGTFITDKTVLDMKAMDSKSNGAIAWSNQTSFTCQDIFKETNATYPSSDVPCDATLTEKSFETDMNLNFQNLSVMGLRILLLKVAGFNLLMTLRLWSS

SEQ ID NO: 103 - protein, 271 aa, Artificial Sequence
  Synthetic
  MISC_FEATURE (122)..(122): Xaa is Ala, Arg, Asn, Asp, Cys, Glu, Gln, Gly, His, Ile, Lys, Met, Phe, Pro, Ser, Thr, Trp, Tyr, or Val.
MRPVTCSVLVLLLMLRRSNGDGDSVTQTEGLVTLTEGLPVMLNCTYQTIYSNPFLFWYVQHLNESPRLLLKSFTDNKRTEHQGFHATLHKSSSSFHLQKSSAQLSDSALYYCALRGNAGAKXTFGGGTRLTVRPDIQNPEPAVYQLKDPRSQDSTLCLFTDFDSQINVPKTMESGTFITDKTVLDMKAMDSKSNGAIAWSNQTSFTCQDIFKETNATYPSSDVPCDATLTEKSFETDMNLNFQNLSVMGLRILLLKVAGFNLLMTLRLWSS

SEQ ID NO: 104 - protein, 271 aa, Artificial Sequence
  Synthetic
  MISC_FEATURE (123)..(123): Xaa is Ala, Arg, Asn, Asp, Cys, Glu, Gln, Gly, His, Ile, Leu, Lys, Met, Phe, Pro, Ser, Trp, Tyr, or Val.
MRPVTCSVLVLLLMLRRSNGDGDSVTQTEGLVTLTEGLPVMLNCTYQTIYSNPFLFWYVQHLNESPRLLLKSFTDNKRTEHQGFHATLHKSSSSFHLQKSSAQLSDSALYYCALRGNAGAKLXFGGGTRLTVRPDIQNPEPAVYQLKDPRSQDSTLCLFTDFDSQINVPKTMESGTFITDKTVLDMKAMDSKSNGAIAWSNQTSFTCQDIFKETNATYPSSDVPCDATLTEKSFETDMNLNFQNLSVMGLRILLLKVAGFNLLMTLRLWSS

SEQ ID NO: 105 - protein, 306 aa, Artificial Sequence
  Synthetic
  MISC_FEATURE (111)..(111): Xaa is Arg, Asn, Asp, Cys, Glu, Gln, Gly, His, Ile, Leu, Lys, Met, Phe, Pro, Ser, Thr, Trp, Tyr, or Val.
MGCRLLSCVAFCLLGIGPLETAVFQTPNYHVTQVGNEVSFNCKQTLGHDTMYWYKQDSKKLLKIMFSYNNKQLIVNETVPRRFSPQSSDKAHLNLRIKSVEPEDSAVYLCXSSSRDWSAETLYFGSGTRLTVLEDLRNVTPPKVSLFEPSKAEIANKQKATLVCLARGFFPDHVELSWWVNGKEVHSGVSTDPQAYKESNYSYCLSSRLRVSATFWHNPRNHFRCQVQFHGLSEEDKWPEGSPKPVTQNISAEAWGRADCGITSASYHQGVLSATILYEILLGKATLYAVLVSGLVLMAMVKKKNS

SEQ ID NO: 106 - protein, 306 aa, Artificial Sequence
  Synthetic
  MISC_FEATURE (112)..(112): Xaa is Ala, Arg, Asn, Asp, Cys, Glu, Gln, Gly, His, Ile, Leu, Lys, Met, Phe, Pro, Thr, Trp, Tyr, or Val.
MGCRLLSCVAFCLLGIGPLETAVFQTPNYHVTQVGNEVSFNCKQTLGHDTMYWYKQDSKKLLKIMFSYNNKQLIVNETVPRRFSPQSSDKAHLNLRIKSVEPEDSAVYLCAXSSRDWSAETLYFGSGTRLTVLEDLRNVTPPKVSLFEPSKAEIANKQKATLVCLARGFFPDHVELSWWVNGKEVHSGVSTDPQAYKESNYSYCLSSRLRVSATFWHNPRNHFRCQVQFHGLSEEDKWPEGSPKPVTQNISAEAWGRADCGITSASYHQGVLSATILYEILLGKATLYAVLVSGLVLMAMVKKKNS

SEQ ID NO: 107 - protein, 306 aa, Artificial Sequence
  Synthetic
  MISC_FEATURE (113)..(113): Xaa is Ala, Arg, Asn, Asp, Cys, Glu, Gln, Gly, His, Ile, Leu, Lys, Met, Phe, Pro, Thr, Trp, Tyr, or Val.
MGCRLLSCVAFCLLGIGPLETAVFQTPNYHVTQVGNEVSFNCKQTLGHDTMYWYKQDSKKLLKIMFSYNNKQLIVNETVPRRFSPQSSDKAHLNLRIKSVEPEDSAVYLCASXSRDWSAETLYFGSGTRLTVLEDLRNVTPPKVSLFEPSKAEIANKQKATLVCLARGFFPDHVELSWWVNGKEVHSGVSTDPQAYKESNYSYCLSSRLRVSATFWHNPRNHFRCQVQFHGLSEEDKWPEGSPKPVTQNISAEAWGRADCGITSASYHQGVLSATILYEILLGKATLYAVLVSGLVLMAMVKKKNS

SEQ ID NO: 108 - protein, 306 aa, Artificial Sequence
  Synthetic
  MISC_FEATURE (114)..(114): Xaa is Ala, Arg, Asn, Asp, Cys, Glu, Gln, Gly, His, Ile, Leu, Lys, Met, Phe, Pro, Thr, Trp, Tyr, or Val.
MGCRLLSCVAFCLLGIGPLETAVFQTPNYHVTQVGNEVSFNCKQTLGHDTMYWYKQDSKKLLKIMFSYNNKQLIVNETVPRRFSPQSSDKAHLNLRIKSVEPEDSAVYLCASSXRDWSAETLYFGSGTRLTVLEDLRNVTPPKVSLFEPSKAEIANKQKATLVCLARGFFPDHVELSWWVNGKEVHSGVSTDPQAYKESNYSYCLSSRLRVSATFWHNPRNHFRCQVQFHGLSEEDKWPEGSPKPVTQNISAEAWGRADCGITSASYHQGVLSATILYEILLGKATLYAVLVSGLVLMAMVKKKNS

SEQ ID NO: 109 - protein, 306 aa, Artificial Sequence
  Synthetic
  MISC_FEATURE (115)..(115): Xaa is Ala, Asn, Asp, Cys, Glu, Gln, Gly, His, Ile, Leu, Lys, Met, Phe, Pro, Ser, Thr, Trp, Tyr, or Val.
MGCRLLSCVAFCLLGIGPLETAVFQTPNYHVTQVGNEVSFNCKQTLGHDTMYWYKQDSKKLLKIMFSYNNKQLIVNETVPRRFSPQSSDKAHLNLRIKSVEPEDSAVYLCASSSXDWSAETLYFGSGTRLTVLEDLRNVTPPKVSLFEPSKAEIANKQKATLVCLARGFFPDHVELSWWVNGKEVHSGVSTDPQAYKESNYSYCLSSRLRVSATFWHNPRNHFRCQVQFHGLSEEDKWPEGSPKPVTQNISAEAWGRADCGITSASYHQGVLSATILYEILLGKATLYAVLVSGLVLMAMVKKKNS

SEQ ID NO: 110 - protein, 306 aa, Artificial Sequence
  Synthetic
  MISC_FEATURE (116)..(116): Xaa is Ala, Arg, Asn, Cys, Glu, Gln, Gly, His, Ile, Leu, Lys, Met, Phe, Pro, Ser, Thr, Trp, Tyr, or Val.
MGCRLLSCVAFCLLGIGPLETAVFQTPNYHVTQVGNEVSFNCKQTLGHDTMYWYKQDSKKLLKIMFSYNNKQLIVNETVPRRFSPQSSDKAHLNLRIKSVEPEDSAVYLCASSSRXWSAETLYFGSGTRLTVLEDLRNVTPPKVSLFEPSKAEIANKQKATLVCLARGFFPDHVELSWWVNGKEVHSGVSTDPQAYKESNYSYCLSSRLRVSATFWHNPRNHFRCQVQFHGLSEEDKWPEGSPKPVTQNISAEAWGRADCGITSASYHQGVLSATILYEILLGKATLYAVLVSGLVLMAMVKKKNS

SEQ ID NO: 111 - protein, 306 aa, Artificial Sequence
  Synthetic
  MISC_FEATURE (117)..(117): Xaa is Ala, Arg, Asn, Asp, Cys, Glu, Gln, Gly, His, Ile, Leu, Lys, Met, Phe, Pro, Ser, Thr, Tyr, or Val.
MGCRLLSCVAFCLLGIGPLETAVFQTPNYHVTQVGNEVSFNCKQTLGHDTMYWYKQDSKKLLKIMFSYNNKQLIVNETVPRRFSPQSSDKAHLNLRIKSVEPEDSAVYLCASSSRDXSAETLYFGSGTRLTVLEDLRNVTPPKVSLFEPSKAEIANKQKATLVCLARGFFPDHVELSWWVNGKEVHSGVSTDPQAYKESNYSYCLSSRLRVSATFWHNPRNHFRCQVQFHGLSEEDKWPEGSPKPVTQNISAEAWGRADCGITSASYHQGVLSATILYEILLGKATLYAVLVSGLVLMAMVKKKNS

SEQ ID NO: 112 - protein, 306 aa, Artificial Sequence
  Synthetic
  MISC_FEATURE (118)..(118): Xaa is Ala, Arg, Asn, Asp, Cys, Glu, Gln, Gly, His, Ile, Leu, Lys, Met, Phe, Pro, Thr, Trp, Tyr, or Val.
MGCRLLSCVAFCLLGIGPLETAVFQTPNYHVTQVGNEVSFNCKQTLGHDTMYWYKQDSKKLLKIMFSYNNKQLIVNETVPRRFSPQSSDKAHLNLRIKSVEPEDSAVYLCASSSRDWXAETLYFGSGTRLTVLEDLRNVTPPKVSLFEPSKAEIANKQKATLVCLARGFFPDHVELSWWVNGKEVHSGVSTDPQAYKESNYSYCLSSRLRVSATFWHNPRNHFRCQVQFHGLSEEDKWPEGSPKPVTQNISAEAWGRADCGITSASYHQGVLSATILYEILLGKATLYAVLVSGLVLMAMVKKKNS

SEQ ID NO: 113 - protein, 306 aa, Artificial Sequence
  Synthetic
  MISC_FEATURE (119)..(119): Xaa is Arg, Asn, Asp, Cys, Glu, Gln, Gly, His, Ile, Leu, Lys, Met, Phe, Pro, Ser, Thr, Trp, Tyr, or Val.
MGCRLLSCVAFCLLGIGPLETAVFQTPNYHVTQVGNEVSFNCKQTLGHDTMYWYKQDSKKLLKIMFSYNNKQLIVNETVPRRFSPQSSDKAHLNLRIKSVEPEDSAVYLCASSSRDWSXETLYFGSGTRLTVLEDLRNVTPPKVSLFEPSKAEIANKQKATLVCLARGFFPDHVELSWWVNGKEVHSGVSTDPQAYKESNYSYCLSSRLRVSATFWHNPRNHFRCQVQFHGLSEEDKWPEGSPKPVTQNISAEAWGRADCGITSASYHQGVLSATILYEILLGKATLYAVLVSGLVLMAMVKKKNS

SEQ ID NO: 114 - protein, 306 aa, Artificial Sequence
  Synthetic
  MISC_FEATURE (120)..(120): Xaa is Ala, Arg, Asn, Asp, Cys, Gln, Gly, His, Ile, Leu, Lys, Met, Phe, Pro, Ser, Thr, Trp, Tyr, or Val.
MGCRLLSCVAFCLLGIGPLETAVFQTPNYHVTQVGNEVSFNCKQTLGHDTMYWYKQDSKKLLKIMFSYNNKQLIVNETVPRRFSPQSSDKAHLNLRIKSVEPEDSAVYLCASSSRDWSAXTLYFGSGTRLTVLEDLRNVTPPKVSLFEPSKAEIANKQKATLVCLARGFFPDHVELSWWVNGKEVHSGVSTDPQAYKESNYSYCLSSRLRVSATFWHNPRNHFRCQVQFHGLSEEDKWPEGSPKPVTQNISAEAWGRADCGITSASYHQGVLSATILYEILLGKATLYAVLVSGLVLMAMVKKKNS

SEQ ID NO: 115 - protein, 306 aa, Artificial Sequence
  Synthetic
  MISC_FEATURE (121)..(121): Xaa is Ala, Arg, Asn, Asp, Cys, Glu, Gln, Gly, His, Ile, Leu, Lys, Met, Phe, Pro, Ser, Trp, Tyr, or Val.
MGCRLLSCVAFCLLGIGPLETAVFQTPNYHVTQVGNEVSFNCKQTLGHDTMYWYKQDSKKLLKIMFSYNNKQLIVNETVPRRFSPQSSDKAHLNLRIKSVEPEDSAVYLCASSSRDWSAEXLYFGSGTRLTVLEDLRNVTPPKVSLFEPSKAEIANKQKATLVCLARGFFPDHVELSWWVNGKEVHSGVSTDPQAYKESNYSYCLSSRLRVSATFWHNPRNHFRCQVQFHGLSEEDKWPEGSPKPVTQNISAEAWGRADCGITSASYHQGVLSATILYEILLGKATLYAVLVSGLVLMAMVKKKNS

SEQ ID NO: 116 - protein, 306 aa, Artificial Sequence
  Synthetic
  MISC_FEATURE (122)..(122): Xaa is Ala, Arg, Asn, Asp, Cys, Glu, Gln, Gly, His, Ile, Lys, Met, Phe, Pro, Ser, Thr, Trp, Tyr, or Val.
MGCRLLSCVAFCLLGIGPLETAVFQTPNYHVTQVGNEVSFNCKQTLGHDTMYWYKQDSKKLLKIMFSYNNKQLIVNETVPRRFSPQSSDKAHLNLRIKSVEPEDSAVYLCASSSRDWSAETXYFGSGTRLTVLEDLRNVTPPKVSLFEPSKAEIANKQKATLVCLARGFFPDHVELSWWVNGKEVHSGVSTDPQAYKESNYSYCLSSRLRVSATFWHNPRNHFRCQVQFHGLSEEDKWPEGSPKPVTQNISAEAWGRADCGITSASYHQGVLSATILYEILLGKATLYAVLVSGLVLMAMVKKKNS

SEQ ID NO: 117 - protein, 306 aa, Artificial Sequence
  Synthetic
  MISC_FEATURE (123)..(123): Xaa is Ala, Arg, Asn, Asp, Cys, Glu, Gln, Gly, His, Ile, Leu, Lys, Met, Phe, Pro, Ser, Thr, Trp, or Val.
MGCRLLSCVAFCLLGIGPLETAVFQTPNYHVTQVGNEVSFNCKQTLGHDTMYWYKQDSKKLLKIMFSYNNKQLIVNETVPRRFSPQSSDKAHLNLRIKSVEPEDSAVYLCASSSRDWSAETLXFGSGTRLTVLEDLRNVTPPKVSLFEPSKAEIANKQKATLVCLARGFFPDHVELSWWVNGKEVHSGVSTDPQAYKESNYSYCLSSRLRVSATFWHNPRNHFRCQVQFHGLSEEDKWPEGSPKPVTQNISAEAWGRADCGITSASYHQGVLSATILYEILLGKATLYAVLVSGLVLMAMVKKKNS

SEQ ID NO: 118 - protein, 23 aa, Homo sapiens
MTEYKLVVVGAGGVGKSALTIQL

SEQ ID NO: 119 - protein, 23 aa, Homo sapiens
MTEYKLVVVGADGVGKSALTIQL

SEQ ID NO: 120 - protein, 23 aa, Homo sapiens
MTEYKLVVVGAVGVGKSALTIQL

SEQ ID NO: 121 - protein, 188 aa, Homo sapiens [sequence omitted]

SEQ ID NO: 122 - protein, 188 aa, Homo sapiens [sequence omitted]

SEQ ID NO: 123 - protein, 188 aa, Homo sapiens
MTEYKLVVVGAVGVGKSALTIQLIQNHFVDEYDPTIEDSYRKQVVIDGETCLLDILDTAGQEEYSAMRDQYMRTGEGFLCVFAINNTKSFEDIHHYREQIKRVKDSEDVPMVLVGNKCDLPSRTVDTKQAQDLARSYGIPFIETSAKTRQGVDDAFYTLVREIRKHKEKMSKDGKKKKKKSKTKCVIM

SEQ ID NO: 124 - protein, 9 aa, Homo sapiens
VVVGADGVG

SEQ ID NO: 125 - protein, 6 aa, Murine
DPNSYY

SEQ ID NO: 126 - protein, 7 aa, Murine
VFSSTEI

SEQ ID NO: 127 - protein, 16 aa, Murine
CAVSGGTNSAGNKLTF

SEQ ID NO: 128 - protein, 5 aa, Murine
LGHDT

SEQ ID NO: 129 - protein, 6 aa, Murine
YNNKQL

SEQ ID NO: 130 - protein, 14 aa, Murine
CASSRDWGPAEQFF

SEQ ID NO: 131 - protein, 137 aa, Murine
MKTVTGPLFLCFWLQLNCVSRGEQVEQRPPHLSVREGDSAVITCTYTDPNSYYFFWYKQEPGASLQLLMKVFSSTEINEGQGFTVLLNKKDKRLSLNLTAAHPGDSAAYFCAVSGGTNSAGNKLTFGIGTRVLVRPD

SEQ ID NO: 132 - protein, 133 aa, Murine
MGCRLLSCVAFCLLGIGPLETAVFQTPNYHVTQVGNEVSFNCKQTLGHDTMYWYKQDSKKLLKIMFSYNNKQLIVNETVPRRFSPQSSDKAHLNLRIKSVEPEDSAVYLCASSRDWGPAEQFFGPGTRLTVLE

SEQ ID NO: 133 - protein, 273 aa, Murine
MKTVTGPLFLCFWLQLNCVSRGEQVEQRPPHLSVREGDSAVITCTYTDPNSYYFFWYKQEPGASLQLLMKVFSSTEINEGQGFTVLLNKKDKRLSLNLTAAHPGDSAAYFCAVSGGTNSAGNKLTFGIGTRVLVRPDIQNPEPAVYQLKDPRSQDSTLCLFTDFDSQINVPKTMESGTFITDKTVLDMKAMDSKSNGAIAWSNQTSFTCQDIFKETNATYPSSDVPCDATLTEKSFETDMNLNFQNLSVMGLRILLLKVAGFNLLMTLRLWSS

SEQ ID NO: 134 - protein, 305 aa, Murine
MGCRLLSCVAFCLLGIGPLETAVFQTPNYHVTQVGNEVSFNCKQTLGHDTMYWYKQDSKKLLKIMFSYNNKQLIVNETVPRRFSPQSSDKAHLNLRIKSVEPEDSAVYLCASSRDWGPAEQFFGPGTRLTVLEDLRNVTPPKVSLFEPSKAEIANKQKATLVCLARGFFPDHVELSWWVNGKEVHSGVSTDPQAYKESNYSYCLSSRLRVSATFWHNPRNHFRCQVQFHGLSEEDKWPEGSPKPVTQNISAEAWGRADCGITSASYHQGVLSATILYEILLGKATLYAVLVSGLVLMAMVKKKNS

SEQ ID NO: 135 - protein, 136 aa, Murine; identical to SEQ ID NO: 13

SEQ ID NO: 136 - protein, 172 aa, Murine; identical to SEQ ID NO: 14

SEQ ID NO: 137 - protein, 6 aa, Murine
NDMFDY

SEQ ID NO: 138 - protein, 7 aa, Murine
VRSNVDK

SEQ ID NO: 139 - protein, 15 aa, Murine
CAAGDSGGSNYKLTF

SEQ ID NO: 140 - protein, 5 aa, Murine
NSHNY

SEQ ID NO: 141 - protein, 6 aa, Murine
SYGAGN

SEQ ID NO: 142 - protein, 14 aa, Murine
CASASWGGYAEQFF

SEQ ID NO: 143 - protein, 141 aa, Murine
MTGFLKALLLVLCLRPEWIKSQQKTGGQQVKQSSPSLTVQEGGILILNCDYENDMFDYFAWYKKYPDNSPTLLISVRSNVDKREDGRFTVFLNKSGKHFSLHITASQPEDTAVYLCAAGDSGGSNYKLTFGKGTLLTVTPN

SEQ ID NO: 144 - protein, 131 aa, Murine
MGSRLFLVLSLLCTKHMEAAVTQSPRNKVTVTGGNVTLSCRQTNSHNYMYWYRQDTGHGLRLIHYSYGAGNLQIGDVPDGYKATRTTQEDFFLLLELASPSQTSLYFCASASWGGYAEQFFGPGTRLTVLE

SEQ ID NO: 145 - protein, 277 aa, Murine
MTGFLKALLLVLCLRPEWIKSQQKTGGQQVKQSSPSLTVQEGGILILNCDYENDMFDYFAWYKKYPDNSPTLLISVRSNVDKREDGRFTVFLNKSGKHFSLHITASQPEDTAVYLCAAGDSGGSNYKLTFGKGTLLTVTPNIQNPEPAVYQLKDPRSQDSTLCLFTDFDSQINVPKTMESGTFITDKTVLDMKAMDSKSNGAIAWSNQTSFTCQDIFKETNATYPSSDVPCDATLTEKSFETDMNLNFQNLSVMGLRILLLKVAGFNLLMTLRLWSS

SEQ ID NO: 146 - protein, 303 aa, Murine
MGSRLFLVLSLLCTKHMEAAVTQSPRNKVTVTGGNVTLSCRQTNSHNYMYWYRQDTGHGLRLIHYSYGAGNLQIGDVPDGYKATRTTQEDFFLLLELASPSQTSLYFCASASWGGYAEQFFGPGTRLTVLEDLRNVTPPKVSLFEPSKAEIANKQKATLVCLARGFFPDHVELSWWVNGKEVHSGVSTDPQAYKESNYSYCLSSRLRVSATFWHNPRNHFRCQVQFHGLSEEDKWPEGSPKPVTQNISAEAWGRADCGITSASYHQGVLSATILYEILLGKATLYAVLVSGLVLMAMVKKKNS

SEQ ID NO: 147 - protein, 136 aa, Murine; identical to SEQ ID NO: 13

SEQ ID NO: 148 - protein, 172 aa, Murine; identical to SEQ ID NO: 14

SEQ ID NO: 149 - protein, 5 aa, Murine
TTMRS

SEQ ID NO: 150 - protein, 5 aa, Murine
LASGT

SEQ ID NO: 151 - protein, 15 aa, Murine
CAADSSNTGYQNFYF

SEQ ID NO: 152 - protein, 5 aa, Murine
SGHLS

SEQ ID NO: 153 - protein, 6 aa, Murine
HYDKME

SEQ ID NO: 154 - protein, 15 aa, Murine
CASSLTDPLDSDYTF

SEQ ID NO: 155 - protein, 133 aa, Murine
MQRNLGAVLGILWVQICWVRGDQVEQSPSALSLHEGTDSALRCNFTTTMRSVQWFRQNSRGSLISLFYLASGTKENGRLKSAFDSKERRYSTLHIRDAQLEDSGTYFCAADSSNTGYQNFYFGKGTSLTVIPN

SEQ ID NO: 156 - protein, 143 aa, Murine
MSNTAFPDPAWNTTLLSWVALFLLGTSSANSGVVQSPRYIIKGKGERSILKCIPISGHLSVAWYQQTQGQELKFFIQHYDKMERDKGNLPSRFSVQQFDDYHSEMNMSALELEDSAVYFCASSLTDPLDSDYTFGSGTRLLVI

SEQ ID NO: 157 - protein, 269 aa, Murine
MQRNLGAVLGILWVQICWVRGDQVEQSPSALSLHEGTDSALRCNFTTTMRSVQWFRQNSRGSLISLFYLASGTKENGRLKSAFDSKERRYSTLHIRDAQLEDSGTYFCAADSSNTGYQNFYFGKGTSLTVIPNIQNPEPAVYQLKDPRSQDSTLCLFTDFDSQINVPKTMESGTFITDKTVLDMKAMDSKSNGAIAWSNQTSFTCQDIFKETNATYPSSDVPCDATLTEKSFETDMNLNFQNLSVMGLRILLLKVAGFNLLMTLRLWSS

SEQ ID NO: 158 - protein, 316 aa, Murine
MSNTAFPDPAWNTTLLSWVALFLLGTSSANSGVVQSPRYIIKGKGERSILKCIPISGHLSVAWYQQTQGQELKFFIQHYDKMERDKGNLPSRFSVQQFDDYHSEMNMSALELEDSAVYFCASSLTDPLDSDYTFGSGTRLLVIEDLRNVTPPKVSLFEPSKAEIANKQKATLVCLARGFFPDHVELSWWVNGKEVHSGVSTDPQAYKESNYSYCLSSRLRVSATFWHNPRNHFRCQVQFHGLSEEDKWPEGSPKPVTQNISAEAWGRADCGITSASYQQGVLSATILYEILLGKATLYAVLVSTLVVMAMVKRKNS

SEQ ID NO: 159 - protein, 136 aa, Murine; identical to SEQ ID NO: 13

SEQ ID NO: 160 - protein, 173 aa, Murine
EDLRNVTPPKVSLFEPSKAEIANKQKATLVCLARGFFPDHVELSWWVNGKEVHSGVSTDPQAYKESNYSYCLSSRLRVSATFWHNPRNHFRCQVQFHGLSEEDKWPEGSPKPVTQNISAEAWGRADCGITSASYQQGVLSATILYEILLGKATLYAVLVSTLVVMAMVKRKNS

SEQ ID NO: 161 - protein, 13 aa, Murine
CAALNTGYQNFYF

SEQ ID NO: 162 - protein, 612 aa, Artificial Sequence
  Synthetic
MQRNLGAVLGILWVQICWVRGDQVEQSPSALSLHEGTDSALRCNFTTTMRSVQWFRQNSRGSLISLFYLASGTKENGRLKSAFDSKERRYSTLHIRDAQLEDSGTYFCAADSSNTGYQNFYFGKGTSLTVIPNIQNPEPAVYQLKDPRSQDSTLCLFTDFDSQINVPKTMESGTFITDKTVLDMKAMDSKSNGAIAWSNQTSFTCQDIFKETNATYPSSDVPCDATLTEKSFETDMNLNFQNLSVMGLRILLLKVAGFNLLMTLRLWSSRAKRSGSGATNFSLLKQAGDVEENPGPMSNTAFPDPAWNTTLLSWVALFLLGTSSANSGVVQSPRYIIKGKGERSILKCIPISGHLSVAWYQQTQGQELKFFIQHYDKMERDKGNLPSRFSVQQFDDYHSEMNMSALELEDSAVYFCASSLTDPLDSDYTFGSGTRLLVIEDLRNVTPPKVSLFEPSKAEIANKQKATLVCLARGFFPDHVELSWWVNGKEVHSGVSTDPQAYKESNYSYCLSSRLRVSATFWHNPRNHFRCQVQFHGLSEEDKWPEGSPKPVTQNISAEAWGRADCGITSASYQQGVLSATILYEILLGKATLYAVLVSTLVVMAMVKRKNS

SEQ ID NO: 163 - DNA, 1839 bp, Artificial Sequence
  Synthetic
atgcagaggaacctgggagctgtgctggggattctgtgggtgcagatttgctgggtgagaggggatcaggtggagcagagtccttcagccctgagcctccacgagggaaccgattctgctctgagatgcaattttacgaccaccatgaggagtgtgcagtggttccgacagaattccaggggcagcctcatcagtttgttctacttggcttcaggaacaaaggagaatgggaggctaaagtcagcatttgattctaaggagcggcgctacagcaccctgcacatcagggatgcccagctggaggactcaggcacttacttctgtgctgctgactcttcgaacacgggttaccagaacttctattttgggaaaggaacaagtttgactgtcattccaaacatccagaacccagaacctgctgtgtaccagttaaaagatcctcggtctcaggacagcaccctctgcctgttcaccgactttgactcccaaatcaatgtgccgaaaaccatggaatctggaacgttcatcactgacaaaactgtgctggacatgaaagctatggattccaagagcaatggggccattgcctggagcaaccagacaagcttcacctgccaagatatcttcaaagagaccaacgccacctaccccagttcagacgttccctgtgatgccacgttgaccgagaaaagctttgaaacagatatgaacctgaactttcaaaacctgtcagttatgggactccgaatcctcctgctgaaagtagcgggatttaacctgctcatgacgctgaggctgtggtccagtcgggccaagcggtccggatccggagccaccaacttcagcctgctgaagcaggccggcgacgtggaggagaaccccggccccatgtctaacactgccttccctgaccccgcctggaacaccaccctgctatcttgggttgctctctttctcctgggaacaagttcagcaaattctggggttgtccagtctccaagatacataatcaaaggaaagggagaaaggtccattctaaaatgtattcccatctctggacatctctctgtggcctggtatcaacagactcaggggcaggaactaaagttcttcattcagcattatgataaaatggagagagataaaggaaacctgcccagcagattctcagtccaacagtttgatgactatcactctgagatgaacatgagtgccttggagctagaggactctgccgtgtacttctgtgccagctctctcacagatccgctagactccgactacaccttcggctcagggaccaggcttttggtaatagaggatctgagaaatgtgactccacccaaggtctccttgtttgagccatcaaaagcagagattgcaaacaaacaaaaggctaccctcgtgtgcttggccaggggcttcttccctgaccacgtggagctgagctggtgggtgaatggcaaggaggtccacagtggggtcagcacggaccctcaggcctacaaggagagcaattatagctactgcctgagcagccgcctgagggtctctgctaccttctggcacaatcctcgcaaccacttccgctgccaagtgcagttccatgggctttcagaggaggacaagtggccagagggctcacccaaacctgtcacacagaacatcagtgcagaggcctggggccgagcagactgtgggattacctcagcatcctatcaacaaggggtcttgtctgccaccatcctctatgagatcctgctagggaaagccaccctgtatgctgtgcttgtcagtacactggtggtgatggctatggtcaaaagaaagaattcatga

SEQ ID NO: 164 - DNA, 15 bp, Artificial Sequence
  Synthetic
accaccatgaggagt

SEQ ID NO: 165 - DNA, 15 bp, Artificial Sequence
  Synthetic
ttggcttcaggaaca

SEQ ID NO: 166 - DNA, 39 bp, Artificial Sequence
  Synthetic
gctgctgactcttcgaacacgggttaccagaacttctat

SEQ ID NO: 167 - DNA, 15 bp, Artificial Sequence
  Synthetic
tctggacatctctct

SEQ ID NO: 168 - DNA, 18 bp, Artificial Sequence
  Synthetic
cattatgataaaatggag

SEQ ID NO: 169 - DNA, 39 bp, Artificial Sequence
  Synthetic
gccagctctctcacagatccgctagactccgactacacc

SEQ ID NO: 170 - DNA, 399 bp, Artificial Sequence
  Synthetic
atgcagaggaacctgggagctgtgctggggattctgtgggtgcagatttgctgggtgagaggggatcaggtggagcagagtccttcagccctgagcctccacgagggaaccgattctgctctgagatgcaattttacgaccaccatgaggagtgtgcagtggttccgacagaattccaggggcagcctcatcagtttgttctacttggcttcaggaacaaaggagaatgggaggctaaagtcagcatttgattctaaggagcggcgctacagcaccctgcacatcagggatgcccagctggaggactcaggcacttacttctgtgctgctgactcttcgaacacgggttaccagaacttctattttgggaaaggaacaagtttgactgtcattccaaac

SEQ ID NO: 171 - DNA, 429 bp, Artificial Sequence
  Synthetic
atgtctaacactgccttccctgaccccgcctggaacaccaccctgctatcttgggttgctctctttctcctgggaacaagttcagcaaattctggggttgtccagtctccaagatacataatcaaaggaaagggagaaaggtccattctaaaatgtattcccatctctggacatctctctgtggcctggtatcaacagactcaggggcaggaactaaagttcttcattcagcattatgataaaatggagagagataaaggaaacctgcccagcagattctcagtccaacagtttgatgactatcactctgagatgaacatgagtgccttggagctagaggactctgccgtgtacttctgtgccagctctctcacagatccgctagactccgactacaccttcggctcagggaccaggcttttggtaata

SEQ ID NO: 172 - DNA, 807 bp, Artificial Sequence
  Synthetic
atgcagaggaacctgggagctgtgctggggattctgtgggtgcagatttgctgggtgagaggggatcaggtggagcagagtccttcagccctgagcctccacgagggaaccgattctgctctgagatgcaattttacgaccaccatgaggagtgtgcagtggttccgacagaattccaggggcagcctcatcagtttgttctacttggcttcaggaacaaaggagaatgggaggctaaagtcagcatttgattctaaggagcggcgctacagcaccctgcacatcagggatgcccagctggaggactcaggcacttacttctgtgctgctgactcttcgaacacgggttaccagaacttctattttgggaaaggaacaagtttgactgtcattccaaacatccagaacccagaacctgctgtgtaccagttaaaagatcctcggtctcaggacagcaccctctgcctgttcaccgactttgactcccaaatcaatgtgccgaaaaccatggaatctggaacgttcatcactgacaaaactgtgctggacatgaaagctatggattccaagagcaatggggccattgcctggagcaaccagacaagcttcacctgccaagatatcttcaaagagaccaacgccacctaccccagttcagacgttccctgtgatgccacgttgaccgagaaaagctttgaaacagatatgaacctgaactttcaaaacctgtcagttatgggactccgaatcctcctgctgaaagtagcgggatttaacctgctcatgacgctgaggctgtggtccagt

SEQ ID NO: 173 - DNA, 951 bp, Artificial Sequence
  Synthetic
atgtctaacactgccttccctgaccccgcctggaacaccaccctgctatcttgggttgctctctttctcctgggaacaagttcagcaaattctggggttgtccagtctccaagatacataatcaaaggaaagggagaaaggtccattctaaaatgtattcccatctctggacatctctctgtggcctggtatcaacagactcaggggcaggaactaaagttcttcattcagcattatgataaaatggagagagataaaggaaacctgcccagcagattctcagtccaacagtttgatgactatcactctgagatgaacatgagtgccttggagctagaggactctgccgtgtacttctgtgccagctctctcacagatccgctagactccgactacaccttcggctcagggaccaggcttttggtaatagaggatctgagaaatgtgactccacccaaggtctccttgtttgagccatcaaaagcagagattgcaaacaaacaaaaggctaccctcgtgtgcttggccaggggcttcttccctgaccacgtggagctgagctggtgggtgaatggcaaggaggtccacagtggggtcagcacggaccctcaggcctacaaggagagcaattatagctactgcctgagcagccgcctgagggtctctgctaccttctggcacaatcctcgcaaccacttccgctgccaagtgcagttccatgggctttcagaggaggacaagtggccagagggctcacccaaacctgtcacacagaacatcagtgcagaggcctggggccgagcagactgtgggattacctcagcatcctatcaacaaggggtcttgtctgccaccatcctctatgagatcctgctagggaaagccaccctgtatgctgtgcttgtcagtacactggtggtgatggctatggtcaaaagaaagaattcatga

SEQ ID NO: 174 - DNA, 408 bp, Artificial Sequence
  Synthetic
atccagaacccagaacctgctgtgtaccagttaaaagatcctcggtctcaggacagcaccctctgcctgttcaccgactttgactcccaaatcaatgtgccgaaaaccatggaatctggaacgttcatcactgacaaaactgtgctggacatgaaagctatggattccaagagcaatggggccattgcctggagcaaccagacaagcttcacctgccaagatatcttcaaagagaccaacgccacctaccccagttcagacgttccctgtgatgccacgttgaccgagaaaagctttgaaacagatatgaacctaaactttcaaaacctgtcagttatgggactccgaatcctcctgctgaaagtagcgggatttaacctgctcatgacgctgaggctgtggtccagt

SEQ ID NO: 175 - DNA, 522 bp, Artificial Sequence
  Synthetic
gaggatctgagaaatgtgactccacccaaggtctccttgtttgagccatcaaaagcagagattgcaaacaaacaaaaggctaccctcgtgtgcttggccaggggcttcttccctgaccacgtggagctgagctggtgggtgaatggcaaggaggtccacagtggggtcagcacggaccctcaggcctacaaggagagcaattatagctactgcctgagcagccgcctgagggtctctgctaccttctggcacaatcctcgcaaccacttccgctgccaagtgcagttccatgggctttcagaggaggacaagtggccagagggctcacccaaacctgtcacacagaacatcagtgcagaggcctggggccgagcagactgtgggattacctcagcatcctatcaacaaggggtcttgtctgccaccatcctctatgagatcctgctagggaaagccaccctgtatgctgtgcttgtcagtacactggtggtgatggctatggtcaaaagaaagaattcatga

SEQ ID NO: 176 - DNA, 1818 bp, Artificial Sequence
  Synthetic
atgaagacggtgactggacctttgttcctgtgcttctggctgcagctgaactgtgtgagcagaggcgagcaggtggagcagcgccctcctcacctgagtgtccgggagggagacagtgccgttatcacctgcacctacacagaccctaacagttattacttcttctggtacaagcaagagccgggggcaagtcttcagttgcttatgaaggttttctcaagtacggaaataaacgaaggacaaggattcactgtcctactgaacaagaaagacaaacgactctctctgaacctcacagctgcccatcctggggactcagccgcgtacttctgcgcagtcagtggagggactaacagtgcagggaacaagctaacttttggaattggaaccagggtgctggtcaggccagacatccagaacccagaacctgctgtgtaccagttaaaagatcctcggtctcaggacagcaccctctgcctgttcaccgactttgactcccaaatcaatgtgccgaaaaccatggaatctggaacgttcatcactgacaaaactgtgctggacatgaaagctatggattccaagagcaatggggccattgcctggagcaaccagacaagcttcacctgccaagatatcttcaaagagaccaacgccacctaccccagttcagacgttccctgtgatgccacgttgaccgagaaaagctttgaaacagatatgaacctaaactttcaaaacctgtcagttatgggactccgaatcctcctgctgaaagtagcgggatttaacctgctcatgacgctgaggctgtggtccagtcgggccaagcggtccggatccggagccaccaacttcagcctgctgaagcaggccggcgacgtggaggagaaccccggccccatgggctgtaggctcctaagctgtgtggccttctgcctcttgggaataggccctttggagacggctgttttccagactccaaactatcatgtcacacaggtgggaaatgaagtgtctttcaattgtaagcaaactctgggccacgatactatgtattggtacaagcaagactctaagaaattgctgaagattatgtttagctacaataataagcaactcattgtaaacgaaacagttccaaggcgcttctcacctcagtcttcagataaagctcatttgaatcttcgaatcaagtctgtagagccggaggactctgctgtgtatctctgtgccagcagtcgggactgggggcctgctgagcagttcttcggaccagggacacgactcaccgtcctagaggatctgagaaatgtgactccacccaaggtctccttgtttgagccatcaaaagcagagattgcaaacaaacaaaaggctaccctcgtgtgcttggccaggggcttcttccctgaccacgtggagctgagctggtgggtgaatggcaaggaggtccacagtggggtcagcacggaccctcaggcctacaaggagagcaattatagctactgcctgagcagccgcctgagggtctctgctaccttctggcacaatcctcgaaaccacttccgctgccaagtgcagttccatgggctttcagaggaggacaagtggccagagggctcacccaaacctgtcacacagaacatcagtgcagaggcctggggccgagcagactgtggaatcacttcagcatcctatcatcagggggttctgtctgcaaccatcctctatgagatcctactggggaaggccaccctatatgctgtgctggtcagtggcctggtgctgatggccatggtcaagaaaaaaaattcctga

SEQ ID NO: 177 - DNA, 18 bp, Artificial Sequence
  Synthetic
gaccctaacagttattac

SEQ ID NO: 178 - DNA, 21 bp, Artificial Sequence
  Synthetic
gttttctcaagtacggaaata

SEQ ID NO: 179 - DNA, 48 bp, Artificial Sequence
  Synthetic
tgcgcagtcagtggagggactaacagtgcagggaacaagctaactttt

SEQ ID NO: 180 - DNA, 15 bp, Artificial Sequence
  Synthetic
ctgggccacgatact

SEQ ID NO: 181 - DNA, 18 bp, Artificial Sequence
  Synthetic
tacaataataagcaactc

SEQ ID NO: 182 - DNA, 42 bp, Artificial Sequence
  Synthetic
tgtgccagcagtcgggactgggggcctgctgagcagttcttc

SEQ ID NO: 183 - DNA, 411 bp, Artificial Sequence
  Synthetic
atgaagacggtgactggacctttgttcctgtgcttctggctgcagctgaactgtgtgagcagaggcgagcaggtggagcagcgccctcctcacctgagtgtccgggagggagacagtgccgttatcacctgcacctacacagaccctaacagttattacttcttctggtacaagcaagagccgggggcaagtcttcagttgcttatgaaggttttctcaagtacggaaataaacgaaggacaaggattcactgtcctactgaacaagaaagacaaacgactctctctgaacctcacagctgcccatcctggggactcagccgcgtacttctgcgcagtcagtggagggactaacagtgcagggaacaagctaacttttggaattggaaccagggtgctggtcaggccagac

SEQ ID NO: 184 - DNA, 399 bp, Artificial Sequence
  Synthetic
atgggctgtaggctcctaagctgtgtggccttctgcctcttgggaataggccctttggagacggctgttttccagactccaaactatcatgtcacacaggtgggaaatgaagtgtctttcaattgtaagcaaactctgggccacgatactatgtattggtacaagcaagactctaagaaattgctgaagattatgtttagctacaataataagcaactcattgtaaacgaaacagttccaaggcgcttctcacctcagtcttcagataaagctcatttgaatcttcgaatcaagtctgtagagccggaggactctgctgtgtatctctgtgccagcagtcgggactgggggcctgctgagcagttcttcggaccagggacacgactcaccgtcctagag

SEQ ID NO: 185 - DNA, 819 bp, Artificial Sequence
  Synthetic
atgaagacggtgactggacctttgttcctgtgcttctggctgcagctgaactgtgtgagcagaggcgagcaggtggagcagcgccctcctcacctgagtgtccgggagggagacagtgccgttatcacctgcacctacacagaccctaacagttattacttcttctggtacaagcaagagccgggggcaagtcttcagttgcttatgaaggttttctcaagtacggaaataaacgaaggacaaggattcactgtcctactgaacaagaaagacaaacgactctctctgaacctcacagctgcccatcctggggactcagccgcgtacttctgcgcagtcagtggagggactaacagtgcagggaacaagctaacttttggaattggaaccagggtgctggtcaggccagacatccagaacccagaacctgctgtgtaccagttaaaagatcctcggtctcaggacagcaccctctgcctgttcaccgactttgactcccaaatcaatgtgccgaaaaccatggaatctggaacgttcatcactgacaaaactgtgctggacatgaaagctatggattccaagagcaatggggccattgcctggagcaaccagacaagcttcacctgccaagatatcttcaaagagaccaacgccacctaccccagttcagacgttccctgtgatgccacgttgaccgagaaaagctttgaaacagatatgaacctaaactttcaaaacctgtcagttatgggactccgaatcctcctgctgaaagtagcgggatttaacctgctcatgacgctgaggctgtggtccagt

SEQ ID NO: 186 - DNA, 918 bp, Artificial Sequence
  Synthetic
atgggctgtaggctcctaagctgtgtggccttctgcctcttgggaataggccctttggagacggctgttttccagactccaaactatcatgtcacacaggtgggaaatgaagtgtctttcaattgtaagcaaactctgggccacgatactatgtattggtacaagcaagactctaagaaattgctgaagattatgtttagctacaataataagcaactcattgtaaacgaaacagttccaaggcgcttctcacctcagtcttcagataaagctcatttgaatcttcgaatcaagtctgtagagccggaggactctgctgtgtatctctgtgccagcagtcgggactgggggcctgctgagcagttcttcggaccagggacacgactcaccgtcctagaggatctgagaaatgtgactccacccaaggtctccttgtttgagccatcaaaagcagagattgcaaacaaacaaaaggctaccctcgtgtgcttggccaggggcttcttccctgaccacgtggagctgagctggtgggtgaatggcaaggaggtccacagtggggtcagcacggaccctcaggcctacaaggagagcaattatagctactgcctgagcagccgcctgagggtctctgctaccttctggcacaatcctcgaaaccacttccgctgccaagtgcagttccatgggctttcagaggaggacaagtggccagagggctcacccaaacctgtcacacagaacatcagtgcagaggcctggggccgagcagactgtggaatcacttcagcatcctatcatcagggggttctgtctgcaaccatcctctatgagatcctactggggaaggccaccctatatgctgtgctggtcagtggcctggtgctgatggccatggtcaagaaaaaaaattcctga

SEQ ID NO: 187 - DNA, 408 bp, Artificial Sequence; identical to SEQ ID NO: 174
  Synthetic

SEQ ID NO: 188 - DNA, 519 bp, Artificial Sequence
  Synthetic
gatctgagaaatgtgactccacccaaggtctccttgtttgagccatcaaaagcagagattgcaaacaaacaaaaggctaccctcgtgtgcttggccaggggcttcttccctgaccacgtggagctgagctggtgggtgaatggcaaggaggtccacagtggggtcagcacggaccctcaggcctacaaggagagcaattatagctactgcctgagcagccgcctgagggtctctgctaccttctggcacaatcctcgaaaccacttccgctgccaagtgcagttccatgggctttcagaggaggacaagtggccagagggctcacccaaacctgtcacacagaacatcagtgcagaggcctggggccgagcagactgtggaatcacttcagcatcctatcatcagggggttctgtctgcaaccatcctctatgagatcctactggggaaggccaccctatatgctgtgctggtcagtggcctggtgctgatggccatggtcaagaaaaaaaattcctga

SEQ ID NO: 189 - DNA, 18 bp, Artificial Sequence
  Synthetic
aatgatatgtttgactat

SEQ ID NO: 190 - DNA, 21 bp, Artificial Sequence
  Synthetic
gtacgctcaaatgtggataag

SEQ ID NO: 191 - DNA, 45 bp, Artificial Sequence
  Synthetic
tgcgcagcaggtgacagtggaggcagcaattacaaactgacattt

SEQ ID NO: 192 - DNA, 15 bp, Artificial Sequence
  Synthetic
aatagccacaactac

SEQ ID NO: 193 - DNA, 18 bp, Artificial Sequence
  Synthetic
tcatatggtgctggcaac

SEQ ID NO: 194 - DNA, 42 bp, Artificial Sequence
  Synthetic
tgtgccagcgcgagctgggggggctatgctgagcagttcttc

SEQ ID NO: 195 - DNA, 423 bp, Artificial Sequence
  Synthetic
atgactggcttcctgaaggccttgctgttggttctgtgcctgcggccagaatggataaagagtcaacagaagactggtggccagcaagttaaacaaagctctccatcgctgactgttcaagagggagggatattgatcctgaattgtgattacgagaatgatatgtttgactattttgcctggtacaaaaaataccctgacaacagccccacactcctgatatccgtacgctcaaatgtggataagagggaagacggaagattcacagttttcttgaacaaaagcggcaaacacttctcactgcacatcacagcctcccagcctgaagacacagcagtgtacctctgcgcagcaggtgacagtggaggcagcaattacaaactgacatttgggaaaggaactctcttaactgtgactccaaac

SEQ ID NO: 196 - DNA, 393 bp, Artificial Sequence
  Synthetic
atgggctccaggctctttctggtcttgagcctcctgtgtacaaaacacatggaggctgcagtcacccaaagccctagaaacaaggtgacagtaacaggaggaaacgtgacattgagctgtcgccagactaatagccacaactacatgtactggtatcggcaggacactgggcatgggctgaggctgatccattactcatatggtgctggcaaccttcaaataggagatgtccctgatgggtacaaggccaccagaacaacgcaagaagacttcttcctcctgctggaattggcttctccctctcagacatctttgtacttctgtgccagcgcgagctgggggggctatgctgagcagttcttcggaccagggacacgactcaccgtcctagag

SEQ ID NO: 197 - DNA, 831 bp, Artificial Sequence
  Synthetic
atgactggcttcctgaaggccttgctgttggttctgtgcctgcggccagaatggataaagagtcaacagaagactggtggccagcaagttaaacaaagctctccatcgctgactgttcaagagggagggatattgatcctgaattgtgattacgagaatgatatgtttgactattttgcctggtacaaaaaataccctgacaacagccccacactcctgatatccgtacgctcaaatgtggataagagggaagacggaagattcacagttttcttgaacaaaagcggcaaacacttctcactgcacatcacagcctcccagcctgaagacacagcagtgtacctctgcgcagcaggtgacagtggaggcagcaattacaaactgacatttgggaaaggaactctcttaactgtgactccaaacatccagaacccagaacctgctgtgtaccagttaaaagatcctcggtctcaggacagcaccctctgcctgttcaccgactttgactcccaaatcaatgtgccgaaaaccatggaatctggaacgttcatcactgacaaaactgtgctggacatgaaagctatggattccaagagcaatggggccattgcctggagcaaccagacaagcttcacctgccaagatatcttcaaagagaccaacgccacctaccccagttcagacgttccctgtgatgccacgttgaccgagaaaagctttgaaacagatatgaacctaaactttcaaaacctgtcagttatgggactccgaatcctcctgctgaaagtagcgggatttaacctgctcatgacgctgaggctgtggtccagt

SEQ ID NO: 198 - DNA, 912 bp, Artificial Sequence
  Synthetic
atgggctccaggctctttctggtcttgagcctcctgtgtacaaaacacatggaggctgcagtcacccaaagccctagaaacaaggtgacagtaacaggaggaaacgtgacattgagctgtcgccagactaatagccacaactacatgtactggtatcggcaggacactgggcatgggctgaggctgatccattactcatatggtgctggcaaccttcaaataggagatgtccctgatgggtacaaggccaccagaacaacgcaagaagacttcttcctcctgctggaattggcttctccctctcagacatctttgtacttctgtgccagcgcgagctgggggggctatgctgagcagttcttcggaccagggacacgactcaccgtcctagaggatctgagaaatgtgactccacccaaggtctccttgtttgagccatcaaaagcagagattgcaaacaaacaaaaggctaccctcgtgtgcttggccaggggcttcttccctgaccacgtggagctgagctggtgggtgaatggcaaggaggtccacagtggggtcagcacggaccctcaggcctacaaggagagcaattatagctactgcctgagcagccgcctgagggtctctgctaccttctggcacaatcctcgaaaccacttccgctgccaagtgcagttccatgggctttcagaggaggacaagtggccagagggctcacccaaacctgtcacacagaacatcagtgcagaggcctggggccgagcagactgtggaatcacttcagcatcctatcatcagggggttctgtctgcaaccatcctctatgagatcctactggggaaggccaccctatatgctgtgctggtcagtggcctggtgctgatggccatggtcaagaaaaaaaattcctga

SEQ ID NO: 199 - DNA, 408 bp, Artificial Sequence; identical to SEQ ID NO: 174
  Synthetic

SEQ ID NO: 200 - DNA, 519 bp, Artificial Sequence; identical to SEQ ID NO: 188
  Synthetic

SEQ ID NO: 201 - protein, 605 aa, Artificial Sequence
  Synthetic
MKTVTGPLFLCFWLQLNCVSRGEQVEQRPPHLSVREGDSAVITCTYTDPNSYYFFWYKQEPGASLQLLMKVFSSTEINEGQGFTVLLNKKDKRLSLNLTAAHPGDSAAYFCAVSGGTNSAGNKLTFGIGTRVLVRPDIQNPEPAVYQLKDPRSQDSTLCLFTDFDSQINVPKTMESGTFITDKTVLDMKAMDSKSNGAIAWSNQTSFTCQDIFKETNATYPSSDVPCDATLTEKSFETDMNLNFQNLSVMGLRILLLKVAGFNLLMTLRLWSSRAKRSGSGATNFSLLKQAGDVEENPGPMGCRLLSCVAFCLLGIGPLETAVFQTPNYHVTQVGNEVSFNCKQTLGHDTMYWYKQDSKKLLKIMFSYNNKQLIVNETVPRRFSPQSSDKAHLNLRIKSVEPEDSAVYLCASSRDWGPAEQFFGPGTRLTVLEDLRNVTPPKVSLFEPSKAEIANKQKATLVCLARGFFPDHVELSWWVNGKEVHSGVSTDPQAYKESNYSYCLSSRLRVSATFWHNPRNHFRCQVQFHGLSEEDKWPEGSPKPVTQNISAEAWGRADCGITSASYHQGVLSATILYEILLGKATLYAVLVSGLVLMAMVKKKNS

SEQ ID NO: 202 - DNA, 1824 bp, Artificial Sequence
  Synthetic
atgactggcttcctgaaggccttgctgttggttctgtgcctgcggccagaatggataaagagtcaacagaagactggtggccagcaagttaaacaaagctctccatcgctgactgttcaagagggagggatattgatcctgaattgtgattacgagaatgatatgtttgactattttgcctggtacaaaaaataccctgacaacagccccacactcctgatatccgtacgctcaaatgtggataagagggaagacggaagattcacagttttcttgaacaaaagcggcaaacacttctcactgcacatcacagcctcccagcctgaagacacagcagtgtacctctgcgcagcaggtgacagtggaggcagcaattacaaactgacatttgggaaaggaactctcttaactgtgactccaaacatccagaacccagaacctgctgtgtaccagttaaaagatcctcggtctcaggacagcaccctctgcctgttcaccgactttgactcccaaatcaatgtgccgaaaaccatggaatctggaacgttcatcactgacaaaactgtgctggacatgaaagctatggattccaagagcaatggggccattgcctggagcaaccagacaagcttcacctgccaagatatcttcaaagagaccaacgccacctaccccagttcagacgttccctgtgatgccacgttgaccgagaaaagctttgaaacagatatgaacctaaactttcaaaacctgtcagttatgggactccgaatcctcctgctgaaagtagcgggatttaacctgctcatgacgctgaggctgtggtccagtcgggccaagcggtccggatccggagccaccaacttcagcctgctgaagcaggccggcgacgtggaggagaaccccggccccatgggctccaggctctttctggtcttgagcctcctgtgtacaaaacacatggaggctgcagtcacccaaagccctagaaacaaggtgacagtaacaggaggaaacgtgacattgagctgtcgccagactaatagccacaactacatgtactggtatcggcaggacactgggcatgggctgaggctgatccattactcatatggtgctggcaaccttcaaataggagatgtccctgatgggtacaaggccaccagaacaacgcaagaagacttcttcctcctgctggaattggcttctccctctcagacatctttgtacttctgtgccagcgcgagctgggggggctatgctgagcagttcttcggaccagggacacgactcaccgtcctagaggatctgagaaatgtgactccacccaaggtctccttgtttgagccatcaaaagcagagattgcaaacaaacaaaaggctaccctcgtgtgcttggccaggggcttcttccctgaccacgtggagctgagctggtgggtgaatggcaaggaggtccacagtggggtcagcacggaccctcaggcctacaaggagagcaattatagctactgcctgagcagccgcctgagggtctctgctaccttctggcacaatcctcgaaaccacttccgctgccaagtgcagttccatgggctttcagaggaggacaagtggccagagggctcacccaaacctgtcacacagaacatcagtgcagaggcctggggccgagcagactgtggaatcacttcagcatcctatcatcagggggttctgtctgcaaccatcctctatgagatcctactggggaaggccaccctatatgctgtgctggtcagtggcctggtgctgatggccatggtcaagaaaaaaaattcctga

SEQ ID NO: 203 - protein, 607 aa, Artificial Sequence
  Synthetic
MTGFLKALLLVLCLRPEWIKSQQKTGGQQVKQSSPSLTVQEGGILILNCDYENDMFDYFAWYKKYPDNSPTLLISVRSNVDKREDGRFTVFLNKSGKHFSLHITASQPEDTAVYLCAAGDSGGSNYKLTFGKGTLLTVTPNIQNPEPAVYQLKDPRSQDSTLCLFTDFDSQINVPKTMESGTFITDKTVLDMKAMDSKSNGAIAWSNQTSFTCQDIFKETNATYPSSDVPCDATLTEKSFETDMNLNFQNLSVMGLRILLLKVAGFNLLMTLRLWSSRAKRSGSGATNFSLLKQAGDVEENPGPMGSRLFLVLSLLCTKHMEAAVTQSPRNKVTVTGGNVTLSCRQTNSHNYMYWYRQDTGHGLRLIHYSYGAGNLQIGDVPDGYKATRTTQEDFFLLLELASPSQTSLYFCASASWGGYAEQFFGPGTRLTVLEDLRNVTPPKVSLFEPSKAEIANKQKATLVCLARGFFPDHVELSWWVNGKEVHSGVSTDPQAYKESNYSYCLSSRLRVSATFWHNPRNHFRCQVQFHGLSEEDKWPEGSPKPVTQNISAEAWGRADCGITSASYHQGVLSATILYEILLGKATLYAVLVSGLVLMAMVKKKNS

SEQ ID NO: 204 - protein, 16 aa, Murine
CAVSGGTNSAGNKLTF

SEQ ID NO: 205 - protein, 14 aa, Murine
CASASWGGYAEQFF

SEQ ID NO: 206 - protein, 14 aa, Murine
CTCSADRGAETLYF

SEQ ID NO: 207 - protein, 15 aa, Murine
  MISC_FEATURE (9)..(9): Wherein X is alanine, arginine, asparagine, asparatic acid, cysteine, glutamic acid, glutamine, histidine, isoleucine, leucine, lysine, methionine, phenylalanine, proline, serine, threonine, tryptophan, tyrosine, or valine
CAADSSNTXYQNFYF

SEQ ID NO: 208 - protein, 133 aa, Murine
  MISC_FEATURE (116)..(116): Wherein X is alanine, arginine, asparagine, asparatic acid, cysteine, glutamic acid, glutamine, histidine, isoleucine, leucine, lysine, methionine, phenylalanine, proline, serine, threonine, tryptophan, tyrosine, or valine
MQRNLGAVLGILWVQICWVRGDQVEQSPSALSLHEGTDSALRCNFTTTMRSVQWFRQNSRGSLISLFYLASGTKENGRLKSAFDSKERRYSTLHIRDAQLEDSGTYFCAADSSNTXYQNFYFGKGTSLTVIPN

SEQ ID NO: 209 - protein, 269 aa, Murine
  MISC_FEATURE (116)..(116): Wherein X is alanine, arginine, asparagine, asparatic acid, cysteine, glutamic acid, glutamine, histidine, isoleucine, leucine, lysine, methionine, phenylalanine, proline, serine, threonine, tryptophan, tyrosine, or valine
MQRNLGAVLGILWVQICWVRGDQVEQSPSALSLHEGTDSALRCNFTTTMRSVQWFRQNSRGSLISLFYLASGTKENGRLKSAFDSKERRYSTLHIRDAQLEDSGTYFCAADSSNTXYQNFYFGKGTSLTVIPNIQNPEPAVYQLKDPRSQDSTLCLFTDFDSQINVPKTMESGTFITDKTVLDMKAMDSKSNGAIAWSNQTSFTCQDIFKETNATYPSSDVPCDATLTEKSFETDMNLNFQNLSVMGLRILLLKVAGFNLLMTLRLWSS